European Patent Application EP 4 610 279 A2, published September 3, 2025. Title: ANTIBODIES SPECIFICALLY BINDING TO MASP-3 FOR THE TREATMENT OF VARIOUS DISEASES AND DISORDERS. Applicant: Omeros Corporation. Application US. The sequence listing filed with the application follows.

SEQUENCE LISTING (313 sequences)

SEQ ID NO: 1 - DNA, 3895 bp, Homo sapiens
  source 1..3895: mol_type = other DNA
attccggcacagggacacaaacaagctcacccaacaaagccaagctgggaggaccaaggccgggcagccgggagcacccaaggcaggaaaatgaggtggctgcttctctattatgctctgtgcttctccctgtcaaaggcttcagcccacaccgtggagctaaacaatatgtttggccagatccagtcgcctggttatccagactcctatcccagtgattcagaggtgacttggaatatcactgtcccagatgggtttcggatcaagctttacttcatgcacttcaacttggaatcctcctacctttgtgaatatgactatgtgaaggtagaaactgaggaccaggtgctggcaaccttctgtggcagggagaccacagacacagagcagactcccggccaggaggtggtcctctcccctggctccttcatgtccatcactttccggtcagatttctccaatgaggagcgtttcacaggctttgatgcccactacatggctgtggatgtggacgagtgcaaggagagggaggacgaggagctgtcctgtgaccactactgccacaactacattggcggctactactgctcctgccgcttcggctacatcctccacacagacaacaggacctgccgagtggagtgcagtgacaacctcttcactcaaaggactggggtgatcaccagccctgacttcccaaacccttaccccaagagctctgaatgcctgtataccatcgagctggaggagggtttcatggtcaacctgcagtttgaggacatatttgacattgaggaccatcctgaggtgccctgcccctatgactacatcaagatcaaagttggtccaaaagttttggggcctttctgtggagagaaagccccagaacccatcagcacccagagccacagtgtcctgatcctgttccatagtgacaactcgggagagaaccggggctggaggctctcatacagggctgcaggaaatgagtgcccagagctacagcctcctgtccatgggaaaatcgagccctcccaagccaagtatttcttcaaagaccaagtgctcgtcagctgtgacacaggctacaaagtgctgaaggataatgtggagatggacacattccagattgagtgtctgaaggatgggacgtggagtaacaagattcccacctgtaaaattgtagactgtagagccccaggagagctggaacacgggctgatcaccttctctacaaggaacaacctcaccacatacaagtctgagatcaaatactcctgtcaggagccctattacaagatgctcaacaataacacaggtatatatacctgttctgcccaaggagtctggatgaataaagtattggggagaagcctacccacctgccttccagagtgtggtcagccctcccgctccctgccaagcctggtcaagaggatcattgggggccgaaatgctgagcctggcctcttcccgtggcaggccctgatagtggtggaggacacttcgagagtgccaaatgacaagtggtttgggagtggggccctgctctctgcgtcctggatcctcacagcagctcatgtgctgcgctcccagcgtagagacaccacggtgataccagtctccaaggagcatgtcaccgtctacctgggcttgcatgatgtgcgagacaaatcgggggcagtcaacagctcagctgcccgagtggtgctccacccagacttcaacatccaaaactacaaccacgatatagctctggtgcagctgcaggagcctgtgcccctgggaccccacgttatgcctgtctgcctgccaaggcttgagcctgaaggcccggccccccacatgctgggcctggtggccggctggggcatctccaatcccaatgtgacagtggatgagatcatcagcagtggcacacggaccttgtcagatgtcctgcagtatgtcaagttacccgtggtgcctcacgctgagtgcaaaactagctatgagtcccgctcgggcaattacagcgtcacggagaacatgttctgtgctggctactacgagggcggcaaagacacgtgccttggagatagcggtggggcctttgtcatctttgatgacttgagccagcgctgggtggtgcaaggcctggtgtcctgggggggacctgaagaatgcggcagcaagcaggtctatggagtctacacaaaggtctccaattacgtggactgggtgtgggagcagatgggcttaccacaaagtgttgtggagccccaggtggaacggtgagctgacttacttcctcggggcctgcctcccctgagcgaagctacaccgcacttccgacagcacactccacattacttatcagaccatatggaatggaacacactgacctagcggtggcttctcctaccgagacagcccccaggaccctgagaggcagagtgtggtatagggaaaaggctccaggcaggagacctgtgttcctgagcttgtccaagtctctttccctgtctgggcctcactctaccgagtaatacaatgcaggagctcaaccaaggcctctgtgccaatcccagcactcctttccaggccatgcttcttaccccagtggcctttattcactcctgaccacttatcaaacccatcggtcctactgttggtataactgagcttggacctgactattagaaaatggtttctaacattgaactgaatgccgcatctgtatattttcctgctctgccttctgggactagccttggcctaatccttcctctaggagaagagcattcaggttttgggagatggctcatagccaagcccctctctcttagtgtgatcccttggagcaccttcatgcctggggtttctctcccaaaagcttcttgcagtctaagccttatcccttatgttccccattaaaggaatttcaaaagacatggagaaagttgggaaggtttgtgctgactgctgggagcagaatagccgtgggaggcccaccaagcccttaaattcccattgtcaactcagaacacatttgggcccatatgccaccctggaacaccagctgacaccatgggcgtccacacctgctgctccagacaagcacaaagcaatctttcagccttgaaatgtattatctgaaaggctacctgaagcccaggcccgaatatggggacttagtcgattacctggaaaaagaaaagacccacactgtgtcctgctgtgcttttgggcaggaaaatggaagaaagagtggggtgggcacattagaagtcacccaaatcctgccaggctgcctggcatccctggggcatgagctgggcggagaatccaccccgcaggatgttcagagggacccactccttcatttttcagagtcaaaggaatcagaggctcacccatggcaggcagtgaaaagagccaggagtcctgggttctagtccctgctctgcccccaactggctgtataacctttgaaaaatcattttctttgtctgagtctctggttctccgtcagcaacaggctggcataaggtcccctgcaggttccttctagctggagcactcagagcttccctgactgctagcagcctctctggccctcacagggctgattgttctccttctccctggagctctctctcctgaaaatctccatcagagcaaggcagccagagaagcccctgagagggaatgattgggaagtgtccactttctcaaccggctcatcaaacacactcctttgtctatgaatggcacatgtaaatgatgttatattttgtatcttttatatcatatgcttcaccattctgtaaagggcctctgcattgttgctcccatcaggggtctcaagtggaaataaaccctcgtggataaccaaaaaaaaaaaaaaaaaaaa

SEQ ID NO: 2 - protein, 728 aa, Homo sapiens
MRWLLLYYALCFSLSKASAHTVELNNMFGQIQSPGYPDSYPSDSEVTWNITVPDGFRIKLYFMHFNLESSYLCEYDYVKVETEDQVLATFCGRETTDTEQTPGQEVVLSPGSFMSITFRSDFSNEERFTGFDAHYMAVDVDECKEREDEELSCDHYCHNYIGGYYCSCRFGYILHTDNRTCRVECSDNLFTQRTGVITSPDFPNPYPKSSECLYTIELEEGFMVNLQFEDIFDIEDHPEVPCPYDYIKIKVGPKVLGPFCGEKAPEPISTQSHSVLILFHSDNSGENRGWRLSYRAAGNECPELQPPVHGKIEPSQAKYFFKDQVLVSCDTGYKVLKDNVEMDTFQIECLKDGTWSNKIPTCKIVDCRAPGELEHGLITFSTRNNLTTYKSEIKYSCQEPYYKMLNNNTGIYTCSAQGVWMNKVLGRSLPTCLPECGQPSRSLPSLVKRIIGGRNAEPGLFPWQALIVVEDTSRVPNDKWFGSGALLSASWILTAAHVLRSQRRDTTVIPVSKEHVTVYLGLHDVRDKSGAVNSSAARVVLHPDFNIQNYNHDIALVQLQEPVPLGPHVMPVCLPRLEPEGPAPHMLGLVAGWGISNPNVTVDEIISSGTRTLSDVLQYVKLPVVPHAECKTSYESRSGNYSVTENMFCAGYYEGGKDTCLGDSGGAFVIFDDLSQRWVVQGLVSWGGPEECGSKQVYGVYTKVSNYVDWVWEQMGLPQSVVEPQVER

SEQ ID NO: 3 - protein, 733 aa, Mus musculus
MRFLSFWRLLLYHALCLALPEVSAHTVELNEMFGQIQSPGYPDSYPSDSEVTWNITVPEGFRIKLYFMHFNLESSYLCEYDYVKVETEDQVLATFCGRETTDTEQTPGQEVVLSPGTFMSVTFRSDFSNEERFTGFDAHYMAVDVDECKEREDEELSCDHYCHNYIGGYYCSCRFGYILHTDNRTCRVECSGNLFTQRTGTITSPDYPNPYPKSSECSYTIDLEEGFMVSLQFEDIFDIEDHPEVPCPYDYIKIKAGSKVWGPFCGEKSPEPISTQTHSVQILFRSDNSGENRGWRLSYRAAGNECPKLQPPVYGKIEPSQAVYSFKDQVLVSCDTGYKVLKDNGVMDTFQIECLKDGAWSNKIPTCKIVDCGAPAGLKHGLVTFSTRNNLTTYKSEIRYSCQQPYYKMLHNTTGVYTCSAHGTWTNEVLKRSLPTCLPVCGQPSRALPNLVKRIIGGRNAELGLFPWQALIVVEDTSRVPNDKWFGSGALLSESWILTAAHVLRSQRRDNTVIPVSKEHVTVYLGLHDVRDKSGAVNSSAARVILHPDFNIQNYNHDIALVQLQKPVPLGAHVMPICLPRPEPEGPAPHMLGLVAGWGISNPNVTVDEIILSGTRTLSDVLQYVKLPVVSHAECKASYESRSGNYSVTENMFCAGYYEGGKDTCLGDSGGAFVIFDEMSQHWVAQGLVSWGGPEECGSKQVYGVYTKVSNYVDWLWEEMNSPRAVRDLQVER

SEQ ID NO: 4 - protein, 733 aa, Rattus norvegicus
MRFLSFRRLLLYHVLCLTLTEVSAHTVELNEMFGQIQSPGYPDSYPSDSEVTWNITVPEGFRVQLYFMHFNLESSYLCEYDYVKVETEDQVLATFCGRETTDTEQTPGQEVVLSPGSFMSVTFRSDFSNEERFTGFDAHYMAVDVDECKEREDEELSCDHYCHNYIGGYYCSCRFGYILHTDNRTCRVECSGNLFTQRTGTITSPDYPNPYPKSSECSYTIDLEEGFMVTLQFEDIFDIEDHPEVPCPYDYIKIKAGSKVWGPFCGEKSPEPISTQSHSIQILFRSDNSGENRGWRLSYRAAGNECPKLQPPVYGKIEPSQAVYSFKDQVLISCDTGYKVLKDNEVMDTFQIECLKDGAWSNKIPTCKIVDCGVPAVLKHGLVTFSTRNNLTTYKSEIRYSCQQPYYKMLHNTTGVYTCSAHGTWTNEVLKRSLPTCLPVCGQPSRALPNLVKRIIGGRNAELGLFPWQALIVVEDTSRIPNDKWFGSGALLSESWILTAAHVLRSQRRDNTVIPVSKDHVTVYLGLHDVRDKSGAVNSSAARVVLHPDFNIQNYNHDIALVQLQEPVPLGAHVMPICLPRPEPEGPAPHMLGLVAGWGISNPNVTVDEIIISGTRTLSDVLQYVKLPVVSHAECKASYESRSGNYSVTENMFCAGYYEGGKDTCLGDSGGAFVIFDEMSQRWVAQGLVSWGGPEECGSKQVYGVYTKVSNYVDWLLEEMNSPRGVRELQVER

SEQ ID NO: 5 - protein, 730 aa, Gallus gallus
MRYPLAWSMCAWLLGVVGAVELTDMFGEIRSPNFPDSYPSDSEVTWNISVPEGFKIKLYYMHFDLESSYLCEYDYVKIEAEDQELATFCGRETTDTEQAPGQQVILSPGPYMGLTFRSDFSNEERFTGFDAHYTAVDVDECLEKSDEELACDHYCHNYIGGYYCSCRFGYILHSDNRTCKVECSDNLYTQRSGVVTSADFPSPYPKSSDCLYRIELEDGFFITLSFEDSFDVEDHPEVTCPYDYIKIKAGQREFGPFCGEKSPGRIETQTNSVQILFHSDNSGENRGWKLSYTAIGNPCPLVQPPINGKIEPSQAKYTFKDQVVISCNTGYKVLKDNLESDSFQIECLKDGTWSNKIPICKIADCQAPPELEHGFVTFLSRNNLTTYRARIQYHCQHPYYHMAPNSTATYTCDASGVWRSEELGTVLPSCRPVCGRPVRALPGIIKRIIGGRNAEPGFFPWQALIVVEDMSRVPNDKWFGSGALLSDSWVLTAAHVLRSQRRDKTVIPVSKEHVTVYLALHDVRNKLEAVNRTVERIILHEDFDIQNYNHDIALVKLKEKVTMGNYVMPICLPQFEHELEGPHPNTLGLVAGWGISNPNITVDEIISSGMRTLSDILQYVKLPVVLHAECKTSYESRSGNYSVTENMFCAGYYEGGKDTCLGDSGGAFVIQDPGTRRWVAQGLVSWGGPEECGSKQVYGVYTKVSNYVDWVEKNTGSSERWTFLDPELER

SEQ ID NO: 6 - protein, 728 aa, Oryctolagus cuniculus
MRWLLLCHALCFSLLKASAHTVELNDMFGQIQSPGYPDSYPSDSEVTWNITVPEGFRIKLYFMHFNLESSYLCEYDYVKVETEDQVLATFCGRETTDTEQTPGQEVVLSPGSFMSITFRSDFSNEERFTGFDAHYMAVDVDECKEREDEELSCDHYCHNYIGGYYCSCRFGYILHTDNRTCRVECSDNLFTQRTGVITSPDYPNPYPKSSECFYTIELEEGFMISLQFEDIFDIEDHPEVPCPYDYIKIKVGENVWGPYCGEKAPEAISTQSHSVQILFRSDNSGENRGWRLSYRAAGNECSELQPPDQGKIEPLQAKYFFKDQVLVSCDTGYKVLKDDVEMDTFQIECLKDGTWSNKIPTCKMVDCGVPAELEHGLLTFSSRSNLTTYASEVTYSCQQPYYRLLHNVSGVYTCSAQGIWTNEVLGRSLPTCIPVCGQPSRSLPSLIKRIIGGRNAEPGLFPWQALIVVEDTSRVPNDKWFGSGALLSESWILTAAHVLRSQRRDNTVIPVSREHVTVYLGLHDVRDKSGAVNSSAARVLLHPDFNIQNYNHDIALVQLQEPVPLGPHVMPICLPRPEPEGPAPYMLGLVAGWGISNPNVTVDEIISSGTRTLSDILQYVKLPVVPHAECKTSYESRSGNYSVTENMFCAGYYEGGKDTCLGDSGGAFVILDDLSRRWVAQGLVSWGGPEECGSKQVYGVYTKVSNYVDWVWEQMGSPQGLGELQVER

SEQ ID NO: 7 - protein, 728 aa, Macaca fascicularis
MRWLLLYHALCFSLSKASAHTVELNDMFGQIQSPGYPDSYPSDSEVTWNITVPDGFRIKLYFMHFNLESSYLCEYDYVKVETEDQVLATFCGRETTDTEQTPGQEVVLSPGSFMSITFRSDFSNEERFTGFDAHYMAVDVDECKEREDEELSCDHYCHNYIGGYYCSCRFGYILHTDNRTCRVECSDNLFTQRTGVITSPDFPNPYPKSSECLYTIELEEGFMVNLQFEDIFDIEDHPEVPCPYDYIKIKVGPKVLGPFCGEKAPEPINTQSHSVLILFHSDNSGENRGWRLSYRAAGNECPELQPPVHGKIEPSQAKYSFKDQVLISCDTGYKVLKDNVEMDTFQIECLKDGTWSNKIPTCKIVDCRAPGELEHGLVTFSTRNNLTTYKSEIRYSCQEPYYKMLNNITGIYTCSAQGVWMNKVLGRSLPTCLPECGQPSRSLPSLVKRIIGGRNAEPGLFPWQALIVVEDTSRVPNDKWFGSGALLSESWILTAAHVLRSQRRDTTVIPVSKEHVTVYLGLHDVRDKSGAVNSSAARVVLHPDFNIQNYNHDIALVQLQEPVPLGPHVMPVCLPRLEPEGPSPHMLGLVAGWGISNPNVTVDEIISSGTRTLSDVLQYVKLPVVPHAECKTSYESRSGNYSVTENMFCAGYYEGGKDTCLGDSGGAFVILDDLSQRWVVQGLVSWGGPEECGSKQVYGVYTKVSNYVDWVWEQMGSPQGRAPGGTVS

SEQ ID NO: 8 - protein, 699 aa, Homo sapiens
MRWLLLYYALCFSLSKASAHTVELNNMFGQIQSPGYPDSYPSDSEVTWNITVPDGFRIKLYFMHFNLESSYLCEYDYVKVETEDQVLATFCGRETTDTEQTPGQEVVLSPGSFMSITFRSDFSNEERFTGFDAHYMAVDVDECKEREDEELSCDHYCHNYIGGYYCSCRFGYILHTDNRTCRVECSDNLFTQRTGVITSPDFPNPYPKSSECLYTIELEEGFMVNLQFEDIFDIEDHPEVPCPYDYIKIKVGPKVLGPFCGEKAPEPISTQSHSVLILFHSDNSGENRGWRLSYRAAGNECPELQPPVHGKIEPSQAKYFFKDQVLVSCDTGYKVLKDNVEMDTFQIECLKDGTWSNKIPTCKIVDCRAPGELEHGLITFSTRNNLTTYKSEIKYSCQEPYYKMLNNNTGIYTCSAQGVWMNKVLGRSLPTCLPVCGLPKFSRKLMARIFNGRPAQKGTTPWIAMLSHLNGQPFCGGSLLGSSWIVTAAHCLHQSLDPKDPTLRDSDLLSPSDFKIILGKHWRLRSDENEQHLGVKHTTLHPKYDPNTFENDVALVELLESPVLNAFVMPICLPEGPQQEGAMVIVSGWGKQFLQRFPETLMEIEIPIVDHSTCQKAYAPLKKKVTRDMICAGEKEGGKDACSGDSGGPMVTLNRERGQWYLVGTVSWGDDCGKKDRYGVYSYIHHNKDWIQRVTGVRN

SEQ ID NO: 9 - protein, 12 aa, synthetic construct
  REGION 1..12: note = Synthetic
VLRSQRRDTTVI

SEQ ID NO: 10 - protein, 15 aa, synthetic construct
  REGION 1..15: note = Synthetic
TAAHVLRSQRRDTTV

SEQ ID NO: 11 - protein, 15 aa, synthetic construct
  REGION 1..15: note = Synthetic
DFNIQNYNHDIALVQ

SEQ ID NO: 12 - protein, 13 aa, synthetic construct
  REGION 1..13: note = Synthetic
PHAECKTSYESRS

SEQ ID NO: 13 - protein, 11 aa, synthetic construct
  REGION 1..11: note = Synthetic
GNYSVTENMFC

SEQ ID NO: 14 - protein, 10 aa, synthetic construct
  REGION 1..10: note = Synthetic
VSNYVDWVWE

SEQ ID NO: 15 - protein, 11 aa, synthetic construct
  REGION 1..11: note = Synthetic
VLRSQRRDTTV

SEQ ID NO: 16 - protein, 13 aa, synthetic construct
  REGION 1..13: note = Synthetic
ECGQPSRSLPSLV

SEQ ID NO: 17 - protein, 11 aa, synthetic construct
  REGION 1..11: note = Synthetic
RNAEPGLFPWQ

SEQ ID NO: 18 - protein, 15 aa, synthetic construct
  REGION 1..15: note = Synthetic
KWFGSGALLSASWIL

SEQ ID NO: 19 - protein, 10 aa, synthetic construct
  REGION 1..10: note = Synthetic
EHVTVYLGLH

SEQ ID NO: 20 - protein, 10 aa, synthetic construct
  REGION 1..10: note = Synthetic
PVPLGPHVMP

SEQ ID NO: 21 - protein, 7 aa, synthetic construct
  REGION 1..7: note = Synthetic
APHMLGL

SEQ ID NO: 22 - protein, 10 aa, synthetic construct
  REGION 1..10: note = Synthetic
SDVLQYVKLP

SEQ ID NO: 23 - protein, 12 aa, synthetic construct
  REGION 1..12: note = Synthetic
AFVIFDDLSQRW

SEQ ID NO: 24 - protein, 114 aa, synthetic construct
  REGION 1..114: note = Synthetic
QVQLKQSGPELVKPGASVKLSCKASGYTFTTDDINWVKQRPGQGLEWIGWIYPRDDRTKYNDKFKDKATLTVDTSSNTAYMDLHSLTSEDSAVYFCSSLEDTYWGQGTLVAVSS

SEQ ID NO: 25 - protein, 114 aa, synthetic construct
  REGION 1..114: note = Synthetic
QVQLKQSGPELVKPGASVKLSCKASGYTFTSNDINWVKQRPGQGLEWIGWIYPRDGSIKYNEKFTDKATLTVDVSSSTAYMELHSLTSEDSAVYFCSGVEDSYWGQGTLVTVSS

SEQ ID NO: 26 - protein, 114 aa, synthetic construct
  REGION 1..114: note = Synthetic
QVQLKQSGPELVKPGASVKLSCKASGYTFTSNDINWVKQRPGQGLEWIGWIYPRDGTTKYNEEFTDKATLTVDVSSSTAFMELHSLTSEDSAVYFCSSVEDSYWGQGTLVTVSS

SEQ ID NO: 27 - protein, 114 aa, synthetic construct
  REGION 1..114: note = Synthetic
QVQLKQSGPELVKPGASVKLSCKASGYTFTSNDINWVKQRPGQGLEWIGWIYPRDGTTKYNEKFTDKATLTVDVSSSTAFMELHRLTSEDSAVYFCSSVEDSYWGQGTLVTVSS

SEQ ID NO: 28 - protein, 116 aa, synthetic construct
  REGION 1..116: note = Synthetic
QIQLVQSGPELKKPGETVKISCKASGYIFTSYGMSWVRQAPGKGLKWMGWINTYSGVPTYADDFKGRFAFSLETSARTPYLQINNLKNEDTATYFCARGGEAMDYWGQGTSVTVSS

SEQ ID NO: 29 - protein, 116 aa, synthetic construct
  REGION 1..116: note = Synthetic
QIQLVQSGPELKTPGETVKISCKASGYIFTSYGITWVKQAPGKGLKWMGWINTYSGVPTYADDFKGRFAFSLETSASTAYLQINNLKNEDTTTYFCTRGGDALDYWGQGTSVTVSS

SEQ ID NO: 30 - protein, 113 aa, synthetic construct
  REGION 1..113: note = Synthetic
QVQLKQSGAELMKPGASVKLSCKATGYTFTGKWIEWVKQRPGHGLEWIGEILPGTGSTNYNEKFKGKATFTADSSSNTAYMQLSSLTTEDSAMYYCLRSEDVWGTGTTVTVSS

SEQ ID NO: 31 - protein, 113 aa, synthetic construct
  REGION 1..113: note = Synthetic
QVQLKQSGAELMKPGASVKLACKATGYTFTGYWIEWIKQRPGQGLEWIGEMLPGSGSTHYNEKFKGKATFTADTSSNTAYMQLSGLTTEDSAIYYCVRSIDYWGQGTTLTVSS

SEQ ID NO: 32 - protein, 125 aa, synthetic construct
  REGION 1..125: note = Synthetic
QVQLKQSGPELARPWASVKISCQAFYTFSRRVHFAIRDTNYWMQWVKQRPGQGLEWIGAIYPGNGDTSYNQKFKGKATLTADKSSSTAYMQLSSLTSEDSAVYYCASGSHYFDYWGQGTTLTVSS

SEQ ID NO: 33 - protein, 123 aa, synthetic construct
  REGION 1..123: note = Synthetic
EVQLQQSGPELVKPGASVKVSCKASGYTLTDYYMNWVKQSHGKSLEWIGDVNPNNDGTTYNQKFKGRATLTVDKSSNTASMELRSLTSEDSAVYYCAICPFYYLGKGTHFDYWGQGTSLTVSS

SEQ ID NO: 34 - protein, 124 aa, synthetic construct
  REGION 1..124: note = Synthetic
EVQLQQSGPVLVKPGASGKMSCKASGYKFTDYYMIWVKQSHGKSLEWIGVIKIYNGGTSYNQKFKGKATLTVDKSSSTAYMELNSLTSEDSAVYYCARGPSLYDYDPYWYFDVWGTGTTVTVSS

SEQ ID NO: 35 - protein, 120 aa, synthetic construct
  REGION 1..120: note = Synthetic
QVQLKQSGTELMKPGASVNLSCKASGYTFTAYWIEWVKQRPGHGLEWIGEILPGSGTTNYNENFKDRATFTADTSSNTAYMQLSSLTSEDSAIYYCARSYYYASRWFAFWGQGTLVTVSS

SEQ ID NO: 36 - protein, 120 aa, synthetic construct
  REGION 1..120: note = Synthetic
EVQLQQPGAELVKPGASVKMSCKASGYTFTSYWITWVKQRPGQGLEWIGDIYPGSGSTNYNEKFKSKATLTVDTSSSTAYMQLSSLTSEDSAVYYCARRRYYATAWFAYWGQGTLVTVSS

SEQ ID NO: 37 - protein, 120 aa, synthetic construct
  REGION 1..120: note = Synthetic
QVQLKQSGAELVRPGASVKLSCKASGYTFTDYYINWVKQRPGQGLEWIARIYPGSGNTYYNEKFKGKATLTAEKSSSTAYMQLSSLTSEDSAVYFCARNYYISSPWFAYWGQGTLVTVSS

SEQ ID NO: 38 - protein, 120 aa, synthetic construct
  REGION 1..120: note = Synthetic
QVQLKQSGAELVTPGASVKMSCKASGYTFTTYPIEWMKQNHGKSLEWIGNFHPYNDDTKYNEKFKGKATLTVEKSSNTVYLELSRLTSDDSAVYFCARRVYYSYFWFGYWGHGTLVTVSS

SEQ ID NO: 39 - protein, 120 aa, synthetic construct
  REGION 1..120: note = Synthetic
QVQLKQSGAELVKPGASVKMSCKASGYTFTTYPIEWMKQNHGKSLEWIGNFHPYNGDSKYNEKFKGKATLTVEKSSSTVYLELSRLPSADSAIYYCARRHYAASPWFAHWGQGTLVTVSS

SEQ ID NO: 40 - protein, 113 aa, synthetic construct
  REGION 1..113: note = Synthetic
DIVMTQSPSSLAVSAGEKVTMTCKSSQSLLNSRTRKNYLAWYQQKPGQSPKLLIYWASTRESGVPDRFTGSGSGTDFSLTISSVQAEDLAVYYCKQSYNLYTFGGGTKLEIKR

SEQ ID NO: 41 - protein, 113 aa, synthetic construct
  REGION 1..113: note = Synthetic
DIVMTQSPSSLAVSAGERVTMSCKSSQSLLISRTRKNYLSWYQQKPGQSPKLLIYWASTRESGVPDRFTGSGSGTDFTLTISSVQAEDLAVYYCKQSYNLYTFGGGTKLEIKR

SEQ ID NO: 42 - protein, 113 aa, synthetic construct
  REGION 1..113: note = Synthetic
DIVMTQSPSSLAVSAGEKVTMSCKSSQSLLISRTRKNYLSWYQQKPGQSPKLLIYWASTRESGVPDRFTGSGSGTDFTLTISSVQAEDLAVYYCKQSYNLYTFGGGTKLEIKR

SEQ ID NO: 43 - protein, 113 aa, synthetic construct
  REGION 1..113: note = Synthetic
DVLMTQTPLTLSVTIGQPASISCKSSQSLLDSDGKTYLNWLLQRPGQSPKRLIYLVSKLDSGVPDRFTGSGSGTDFTLKISRVEAEDLGVYYCWQGTHFPWTFGGGTKLEIKR

SEQ ID NO: 44 - protein, 113 aa, synthetic construct
  REGION 1..113: note = Synthetic
DIVMTQAPLTLSVTIGQPASISCKSSQSLLDSDGKTYLSWLLQRPGQSPKRLIYLVSKLDSGVPDRFTGSGSGTDFTLKISRVEAEDLGVYYCWQGTHFPYTFGGGTKLEIKR

SEQ ID NO: 45 - protein, 113 aa, synthetic construct
  REGION 1..113: note = Synthetic
DIVMTQSPSSLAVSAGEKVTMSCKSSQSLLNSRTRKNYLAWYQQKPGQSPKLLIYWASTRESGVPDRFTGSGSGTDFTLTISSVQAEDLAVYYCKQSYNIPTFGGGTKLEIKR

SEQ ID NO: 46 - protein, 113 aa, synthetic construct
  REGION 1..113: note = Synthetic
DVLMTQTPLSLPVSLGEQASISCRSSQSLVQSNGNTYLHWYLQKPGQSPKLLIYKVSNRFSGVPDRFSGSGSGTDFTLKISRVEAEDLGVYFCSQSTHVPPTFGGGTKLEIKR

SEQ ID NO: 47 - protein, 108 aa, synthetic construct
  REGION 1..108: note = Synthetic
DIQLTQSPAILSVSPGERVSFSCRASQSIGTSIHWYQQRTNGSPRLLIKYASESISGIPSRFSGSGSGTDFTLSINSVESEDIADYYCQQSNSWPYTFGGGTKLEIKR

SEQ ID NO: 48 - protein, 108 aa, synthetic construct
  REGION 1..108: note = Synthetic
DIQMTQTPASLSASLGDRVTISCRASQDISNFLNWYQQKPNGTVKLLVFYTSRLHSGVPSRFSGSGSGAEHSLTISNLEQEDVATYFCQQGFTLPWTFGGGTKVEIKR

SEQ ID NO: 49 - protein, 113 aa, synthetic construct
  REGION 1..113: note = Synthetic
DVLMTQTPLSLPVSLGDQASFSCRSSQSLIHSNGNTYLHWYLQKPGQSPKLLIYKVSNRFSGVPDRFSGSGSGTDFTLKISRVEAEDLGVYFCSQSTHVPWTFGGGTKLEIKR

SEQ ID NO: 50 - protein, 108 aa, synthetic construct
  REGION 1..108: note = Synthetic
DIVMTQSQKFMSTSIGDRVSVTCRASQNVGPNLAWYQQKPGQSPKALIYSASYRFSGVPDRFTGSGSGTDFTLTISNVQSEDLAEYFCQQYNRYPFTFGSGTKLEIKR

SEQ ID NO: 51 - protein, 108 aa, synthetic construct
  REGION 1..108: note = Synthetic
DIVMTQSQKFMSTSVGDRVSITCKASQNVGTAVAWYQQKPGQSPKLLISSASNRYTGVPDRFTGSGSGTDFTLTISNMQSEDVADYFCQQYNSYPLTFGAGTKLELKR

SEQ ID NO: 52 - protein, 108 aa, synthetic construct
  REGION 1..108: note = Synthetic
DIVMTQSQKFMSTSVGDRVSVTCKASQNVGPNVAWYQQKPGQSPKALIYSASYRYSGVPDRFTGSGSGTDFTLTISNVQSEDLADYFCQQYNRYPLTFGAGTKLELKR

SEQ ID NO: 53 - protein, 110 aa, synthetic construct
  REGION 1..110: note = Synthetic
DIVMTQSQKFMSTSVGDRVNVTCKASQNVGTHVAWYQQKPGQSPKALIYSASYRYSGVPDRFTGSGSGTDFTLTISNVQSEDLAEYFCQQYNSYPRALTFGAGTKLELKR

SEQ ID NO: 54 - protein, 108 aa, synthetic construct
  REGION 1..108: note = Synthetic
DIVMTQSQKFMSTSVGDRVNVTCKASQNVGPTVAWYQQKPGQSPKALIYSASYRYSGVPDRFTGSGSGTDFTLTISNVHSEDLAEYFCQQYNSYPFTFGSGTKLEIKR

SEQ ID NO: 55 - protein, 30 aa, synthetic construct
  REGION 1..30: note = Synthetic
QVQLKQSGPELVKPGASVKLSCKASGYTFT

SEQ ID NO: 56 - protein, 5 aa, synthetic construct
  REGION 1..5: note = Synthetic
TDDIN

SEQ ID NO: 57 - protein, 14 aa, synthetic construct
  REGION 1..14: note = Synthetic
WVKQRPGQGLEWIG

SEQ ID NO: 58 - protein, 17 aa, synthetic construct
  REGION 1..17: note = Synthetic
WIYPRDDRTKYNDKFKD

SEQ ID NO: 59 - protein, 32 aa, synthetic construct
  REGION 1..32: note = Synthetic
KATLTVDTSSNTAYMDLHSLTSEDSAVYFCSS

SEQ ID NO: 60 - protein, 5 aa, synthetic construct
  REGION 1..5: note = Synthetic
LEDTY

SEQ ID NO: 61 - protein, 11 aa, synthetic construct
  REGION 1..11: note = Synthetic
WGQGTLVAVSS

SEQ ID NO: 62 - protein, 5 aa, synthetic construct
  REGION 1..5: note = Synthetic
SNDIN

SEQ ID NO: 63 - protein, 17 aa, synthetic construct
  REGION 1..17: note = Synthetic
WIYPRDGSIKYNEKFTD

SEQ ID NO: 64 - protein, 32 aa, synthetic construct
  REGION 1..32: note = Synthetic
KATLTVDVSSSTAYMELHSLTSEDSAVYFCSG

SEQ ID NO: 65 - protein, 5 aa, synthetic construct
  REGION 1..5: note = Synthetic
VEDSY

SEQ ID NO: 66 - protein, 11 aa, synthetic construct
  REGION 1..11: note = Synthetic
WGQGTLVTVSS

SEQ ID NO: 67 - protein, 17 aa, synthetic construct
  REGION 1..17: note = Synthetic
WIYPRDGTTKYNEEFTD

SEQ ID NO: 68 - protein, 32 aa, synthetic construct
  REGION 1..32: note = Synthetic
KATLTVDVSSSTAFMELHSLTSEDSAVYFCSS

SEQ ID NO: 69 - protein, 17 aa, synthetic construct
  REGION 1..17: note = Synthetic
WIYPRDGTTKYNEKFTD

SEQ ID NO: 70 - protein, 32 aa, synthetic construct
  REGION 1..32: note = Synthetic
KATLTVDVSSSTAFMELHRLTSEDSAVYFCSS

SEQ ID NO: 71 - protein, 30 aa, synthetic construct
  REGION 1..30: note = Synthetic
QIQLVQSGPELKKPGETVKISCKASGYIFT

SEQ ID NO: 72 - protein, 5 aa, synthetic construct
  REGION 1..5: note = Synthetic
SYGMS

SEQ ID NO: 73 - protein, 14 aa, synthetic construct
  REGION 1..14: note = Synthetic
WVRQAPGKGLKWMG

SEQ ID NO: 74 - protein, 17 aa, synthetic construct
  REGION 1..17: note = Synthetic
WINTYSGVPTYADDFKG

SEQ ID NO: 75 - protein, 32 aa, synthetic construct
  REGION 1..32: note = Synthetic
RFAFSLETSARTPYLQINNLKNEDTATYFCAR

SEQ ID NO: 76 - protein, 7 aa, synthetic construct
  REGION 1..7: note = Synthetic
GGEAMDY

SEQ ID NO: 77 - protein, 11 aa, synthetic construct
  REGION 1..11: note = Synthetic
WGQGTSVTVSS

SEQ ID NO: 78 - protein, 30 aa, synthetic construct
  REGION 1..30: note = Synthetic
QIQLVQSGPELKTPGETVKISCKASGYIFT

SEQ ID NO: 79 - protein, 5 aa, synthetic construct
  REGION 1..5: note = Synthetic
SYGIT

SEQ ID NO: 80 - protein, 14 aa, synthetic construct
  REGION 1..14: note = Synthetic
WVKQAPGKGLKWMG

SEQ ID NO: 81 - protein, 32 aa, synthetic construct
  REGION 1..32: note = Synthetic
RFAFSLETSASTAYLQINNLKNEDTTTYFCTR

SEQ ID NO: 82 - protein, 7 aa, synthetic construct
  REGION 1..7: note = Synthetic
GGDALDY

SEQ ID NO: 83 - protein, 30 aa, synthetic construct
  REGION 1..30: note = Synthetic
QVQLKQSGAELMKPGASVKLSCKATGYTFT

SEQ ID NO: 84 - protein, 5 aa, synthetic construct
  REGION 1..5: note = Synthetic
GKWIE

SEQ ID NO: 85 - protein, 14 aa, synthetic construct
  REGION 1..14: note = Synthetic
WVKQRPGHGLEWIG

SEQ ID NO: 86 - protein, 17 aa, synthetic construct
  REGION 1..17: note = Synthetic
EILPGTGSTNYNEKFKG

SEQ ID NO: 87 - protein, 32 aa, synthetic construct
  REGION 1..32: note = Synthetic
KATFTADSSSNTAYMQLSSLTTEDSAMYYCLR

SEQ ID NO: 88 - protein, 4 aa, synthetic construct
  REGION 1..4: note = Synthetic
SEDV

SEQ ID NO: 89 - protein, 11 aa, synthetic construct
  REGION 1..11: note = Synthetic
WGTGTTVTVSS

SEQ ID NO: 90 - protein, 30 aa, synthetic construct
  REGION 1..30: note = Synthetic
QVQLKQSGAELMKPGASVKLACKATGYTFT

SEQ ID NO: 91 - protein, 5 aa, synthetic construct
  REGION 1..5: note = Synthetic
GYWIE

SEQ ID NO: 92 - protein, 14 aa, synthetic construct
  REGION 1..14: note = Synthetic
WIKQRPGQGLEWIG

SEQ ID NO: 93 - protein, 17 aa, synthetic construct
  REGION 1..17: note = Synthetic
EMLPGSGSTHYNEKFKG

SEQ ID NO: 94 - protein, 32 aa, synthetic construct
  REGION 1..32: note = Synthetic
KATFTADTSSNTAYMQLSGLTTEDSAIYYCVR

SEQ ID NO: 95 - protein, 4 aa, synthetic construct
  REGION 1..4: note = Synthetic
SIDY

SEQ ID NO: 96 - protein, 11 aa, synthetic construct
  REGION 1..11: note = Synthetic
WGQGTTLTVSS

SEQ ID NO: 97 - protein, 30 aa, synthetic construct
  REGION 1..30: note = Synthetic
EVQLQQPGAELVKPGASVKMSCKASGYTFT

SEQ ID NO: 98 - protein, 5 aa, synthetic construct
  REGION 1..5: note = Synthetic
SYWIT

SEQ ID NO: 99 - protein, 17 aa, synthetic construct
  REGION 1..17: note = Synthetic
DIYPGSGSTNYNEKFKS

SEQ ID NO: 100 - protein, 32 aa, synthetic construct
  REGION 1..32: note = Synthetic
KATLTVDTSSSTAYMQLSSLTSEDSAVYYCAR

SEQ ID NO: 101 - protein, 11 aa, synthetic construct
  REGION 1..11: note = Synthetic
RRYYATAWFAY

SEQ ID NO: 102 - protein, 30 aa, synthetic construct
  REGION 1..30: note = Synthetic
QVQLKQSGAELVRPGASVKLSCKASGYTFT

SEQ ID NO: 103 - protein, 5 aa, synthetic construct
  REGION 1..5: note = Synthetic
DYYIN

SEQ ID NO: 104 - protein, 14 aa, synthetic construct
  REGION 1..14: note = Synthetic
WVKQRPGQGLEWIA

SEQ ID NO: 105 - protein, 17 aa, synthetic construct
  REGION 1..17: note = Synthetic
RIYPGSGNTYYNEKFKG

SEQ ID NO: 106 - protein, 32 aa, synthetic construct
  REGION 1..32: note = Synthetic
KATLTAEKSSSTAYMQLSSLTSEDSAVYFCAR

SEQ ID NO: 107 - protein, 11 aa, synthetic construct
  REGION 1..11: note = Synthetic
NYYISSPWFAY

SEQ ID NO: 108 - protein, 30 aa, synthetic construct
  REGION 1..30: note = Synthetic
QVQLKQSGPELARPWASVKISCQAFYTFSR

SEQ ID NO: 109 - protein, 14 aa, synthetic construct
  REGION 1..14: note = Synthetic
RVHFAIRDTNYWMQ

SEQ ID NO: 110 - protein, 17 aa, synthetic construct
  REGION 1..17: note = Synthetic
AIYPGNGDTSYNQKFKG

SEQ ID NO: 111 - protein, 32 aa, synthetic construct
  REGION 1..32: note = Synthetic
KATLTADKSSSTAYMQLSSLTSEDSAVYYCAS

SEQ ID NO: 112 - protein, 7 aa, synthetic construct
  REGION 1..7: note = Synthetic
GSHYFDY

SEQ ID NO: 113 - protein, 30 aa, synthetic construct
  REGION 1..30: note = Synthetic
QVQLKQSGAELVTPGASVKMSCKASGYTFT

SEQ ID NO: 114 - protein, 5 aa, synthetic construct
  REGION 1..5: note = Synthetic
TYPIE

SEQ ID NO: 115 - protein, 14 aa, synthetic construct
  REGION 1..14: note = Synthetic
WMKQNHGKSLEWIG

SEQ ID NO: 116 - protein, 17 aa, synthetic construct
  REGION 1..17: note = Synthetic
NFHPYNDDTKYNEKFKG

SEQ ID NO: 117 - protein, 32 aa, synthetic construct
  REGION 1..32: note = Synthetic
KATLTVEKSSNTVYLELSRLTSDDSAVYFCAR

SEQ ID NO: 118 - protein, 11 aa, synthetic construct
  REGION 1..11: note = Synthetic
RVYYSYFWFGY

SEQ ID NO: 119 - protein, 11 aa, synthetic construct
  REGION 1..11: note = Synthetic
WGHGTLVTVSS

SEQ ID NO: 120 - protein, 30 aa, synthetic construct
  REGION 1..30: note = Synthetic
QVQLKQSGAELVKPGASVKMSCKASGYTFT

SEQ ID NO: 121 - protein, 17 aa, synthetic construct
  REGION 1..17: note = Synthetic
NFHPYNGDSKYNEKFKG

SEQ ID NO: 122 - protein, 32 aa, synthetic construct
  REGION 1..32: note = Synthetic
KATLTVEKSSSTVYLELSRLPSADSAIYYCAR

SEQ ID NO: 123 - protein, 11 aa, synthetic construct
  REGION 1..11: note = Synthetic
RHYAASPWFAH

SEQ ID NO: 124 - protein, 30 aa, synthetic construct
  REGION 1..30: note = Synthetic
EVQLQQSGPELVKPGASVKVSCKASGYTLT

SEQ ID NO: 125 - protein, 5 aa, synthetic construct
  REGION 1..5: note = Synthetic
DYYMN

SEQ ID NO: 126 - protein, 14 aa, synthetic construct
  REGION 1..14: note = Synthetic
WVKQSHGKSLEWIG

SEQ ID NO: 127 - protein, 17 aa, synthetic construct
  REGION 1..17: note = Synthetic
DVNPNNDGTTYNQKFKG

SEQ ID NO: 128 - protein, 32 aa, synthetic construct
  REGION 1..32: note = Synthetic
RATLTVDKSSNTASMELRSLTSEDSAVYYCAI

SEQ ID NO: 129 - protein, 14 aa, synthetic construct
  REGION 1..14: note = Synthetic
CPFYYLGKGTHFDY

SEQ ID NO: 130 - protein, 11 aa, synthetic construct
  REGION 1..11: note = Synthetic
WGQGTSLTVSS

SEQ ID NO: 131 - protein, 30 aa, synthetic construct
  REGION 1..30: note = Synthetic
EVQLQQSGPVLVKPGASGKMSCKASGYKFT

SEQ ID NO: 132 - protein, 5 aa, synthetic construct
  REGION 1..5: note = Synthetic
DYYMI

SEQ ID NO: 133 - protein, 17 aa, synthetic construct
  REGION 1..17: note = Synthetic
VIKIYNGGTSYNQKFKG

SEQ ID NO: 134 - protein, 32 aa, synthetic construct
  REGION 1..32: note = Synthetic
KATLTVDKSSSTAYMELNSLTSEDSAVYYCAR

SEQ ID NO: 135 - protein, 15 aa, synthetic construct
  REGION 1..15: note = Synthetic
GPSLYDYDPYWYFDV

SEQ ID NO: 136 - protein, 30 aa, synthetic construct
  REGION 1..30: note = Synthetic
QVQLKQSGTELMKPGASVNLSCKASGYTFT

SEQ ID NO: 137 - protein, 5 aa, synthetic construct
  REGION 1..5: note = Synthetic
AYWIE

SEQ ID NO: 138 - protein, 17 aa, synthetic construct
  REGION 1..17: note = Synthetic
EILPGSGTTNYNENFKD

SEQ ID NO: 139 - protein, 32 aa, synthetic construct
  REGION 1..32: note = Synthetic
RATFTADTSSNTAYMQLSSLTSEDSAIYYCAR

SEQ ID NO: 140 - protein, 11 aa, synthetic construct
  REGION 1..11: note = Synthetic
SYYYASRWFAF

SEQ ID NO: 141 - protein, 23 aa, synthetic construct
  REGION 1..23: note = Synthetic
DIVMTQSPSSLAVSAGEKVTMTC

SEQ ID NO: 142 - protein, 17 aa, synthetic construct
  REGION 1..17: note = Synthetic
KSSQSLLNSRTRKNYLA

SEQ ID NO: 143 - protein, 15 aa, synthetic construct
  REGION 1..15: note = Synthetic
WYQQKPGQSPKLLIY

SEQ ID NO: 144 - protein, 7 aa, synthetic construct
  REGION 1..7: note = Synthetic
WASTRES

SEQ ID NO: 145 - protein, 32 aa, synthetic construct
  REGION 1..32: note = Synthetic
GVPDRFTGSGSGTDFSLTISSVQAEDLAVYYC

SEQ ID NO: 146 - protein, 8 aa, synthetic construct
  REGION 1..8: note = Synthetic
KQSYNLYT

SEQ ID NO: 147 - protein, 11 aa, synthetic construct
  REGION 1..11: note = Synthetic
FGGGTKLEIKR

SEQ ID NO: 148 - protein, 23 aa, synthetic construct
  REGION 1..23: note = Synthetic
DIVMTQSPSSLAVSAGERVTMSC

SEQ ID NO: 149 - protein, 17 aa, synthetic construct
  REGION 1..17: note = Synthetic
KSSQSLLISRTRKNYLS

SEQ ID NO: 150 - protein, 32 aa, synthetic construct
  REGION 1..32: note = Synthetic
GVPDRFTGSGSGTDFTLTISSVQAEDLAVYYC

SEQ ID NO: 151 - protein, 23 aa, synthetic construct
  REGION 1..23: note = Synthetic
DIVMTQSPSSLAVSAGEKVTMSC

SEQ ID NO: 152 - protein, 23 aa, synthetic construct
  REGION 1..23: note = Synthetic
DVLMTQTPLTLSVTIGQPASISC

SEQ ID NO: 153 - protein, 16 aa, synthetic construct
  REGION 1..16: note = Synthetic
KSSQSLLDSDGKTYLN

SEQ ID NO: 154 - protein, 15 aa, synthetic construct
  REGION 1..15: note = Synthetic
WLLQRPGQSPKRLIY

SEQ ID NO: 155 - protein, 7 aa, synthetic construct
  REGION 1..7: note = Synthetic
LVSKLDS

SEQ ID NO: 156 - protein, 32 aa, synthetic construct
  REGION 1..32: note = Synthetic
GVPDRFTGSGSGTDFTLKISRVEAEDLGVYYC

SEQ ID NO: 157 - protein, 9 aa, synthetic construct
  REGION 1..9: note = Synthetic
WQGTHFPWT

SEQ ID NO: 158 - protein, 23 aa, synthetic construct
  REGION 1..23: note = Synthetic
DIVMTQAPLTLSVTIGQPASISC

SEQ ID NO: 159 - protein, 16 aa, synthetic construct
  REGION 1..16: note = Synthetic
KSSQSLLDSDGKTYLS

SEQ ID NO: 160 - protein, 9 aa, synthetic construct
  REGION 1..9: note = Synthetic
WQGTHFPYT

SEQ ID NO: 161 - protein, 8 aa, synthetic construct
  REGION 1..8: note = Synthetic
KQSYNIPT

SEQ ID NO: 162 - protein, 23 aa, synthetic construct
  REGION 1..23: note = Synthetic
DVLMTQTPLSLPVSLGEQASISC

SEQ ID NO: 163 - protein, 16 aa, synthetic construct
  REGION 1..16: note = Synthetic
RSSQSLVQSNGNTYLH

SEQ ID NO: 164 - protein, 15 aa, synthetic construct
  REGION 1..15: note = Synthetic
WYLQKPGQSPKLLIY

SEQ ID NO: 165 - protein, 7 aa, synthetic construct
  REGION 1..7: note = Synthetic
KVSNRFS

SEQ ID NO: 166 - protein, 32 aa, synthetic construct
  REGION 1..32: note = Synthetic
GVPDRFSGSGSGTDFTLKISRVEAEDLGVYFC

SEQ ID NO: 167 - protein, 9 aa, synthetic construct
  REGION 1..9: note = Synthetic
SQSTHVPPT

SEQ ID NO: 168 - protein, 23 aa, synthetic construct
  REGION 1..23: note = Synthetic
DIVMTQSQKFMSTSVGDRVSITC

SEQ ID NO: 169 - protein, 11 aa, synthetic construct
  REGION 1..11: note = Synthetic
KASQNVGTAVA

SEQ ID NO: 170 - protein, 15 aa, synthetic construct
  REGION 1..15: note = Synthetic
WYQQKPGQSPKLLIS

SEQ ID NO: 171 - protein, 7 aa, synthetic construct
  REGION 1..7: note = Synthetic
SASNRYT

SEQ ID NO: 172 - protein, 32 aa, synthetic construct
  REGION 1..32: note = Synthetic
GVPDRFTGSGSGTDFTLTISNMQSEDVADYFC

SEQ ID NO: 173 - protein, 9 aa, synthetic construct
  REGION 1..9: note = Synthetic
QQYNSYPLT

SEQ ID NO: 174 - protein, 11 aa, synthetic construct
  REGION 1..11: note = Synthetic
FGAGTKLELKR

SEQ ID NO: 175 - protein, 23 aa, synthetic construct
  REGION 1..23: note = Synthetic
DIVMTQSQKFMSTSVGDRVSVTC

SEQ ID NO: 176 - protein, 11 aa, synthetic construct
  REGION 1..11: note = Synthetic
KASQNVGPNVA

SEQ ID NO: 177 - protein, 15 aa, synthetic construct
  REGION 1..15: note = Synthetic
WYQQKPGQSPKALIY

SEQ ID NO: 178 - protein, 7 aa, synthetic construct
  REGION 1..7: note = Synthetic
SASYRYS

SEQ ID NO: 179 - protein, 32 aa, synthetic construct
  REGION 1..32: note = Synthetic
GVPDRFTGSGSGTDFTLTISNVQSEDLADYFC

SEQ ID NO: 180 - protein, 9 aa, synthetic construct
  REGION 1..9: note = Synthetic
QQYNRYPLT

SEQ ID NO: 181 - protein, 23 aa, synthetic construct
  REGION 1..23: note = Synthetic
DIQLTQSPAILSVSPGERVSFSC

SEQ ID NO: 182 - protein, 11 aa, synthetic construct
  REGION 1..11: note = Synthetic
RASQSIGTSIH

SEQ ID NO: 183 - protein, 15 aa, synthetic construct
  REGION 1..15: note = Synthetic
WYQQRTNGSPRLLIK

SEQ ID NO: 184 - protein, 7 aa, synthetic construct
  REGION 1..7: note = Synthetic
YASESIS

SEQ ID NO: 185 - protein, 32 aa, synthetic construct
  REGION 1..32: note = Synthetic
GIPSRFSGSGSGTDFTLSINSVESEDIADYYC

SEQ ID NO: 186 - protein, 9 aa, synthetic construct
  REGION 1..9: note = Synthetic
QQSNSWPYT

SEQ ID NO: 187 - protein, 23 aa, synthetic construct
  REGION 1..23: note = Synthetic
DIVMTQSQKFMSTSVGDRVNVTC

SEQ ID NO: 188 - protein, 11 aa, synthetic construct
  REGION 1..11: note = Synthetic
KASQNVGTHVA

SEQ ID NO: 189 - protein, 32 aa, synthetic construct
  REGION 1..32: note = Synthetic
GVPDRFTGSGSGTDFTLTISNVQSEDLAEYFC

SEQ ID NO: 190 - protein, 11 aa, synthetic construct
  REGION 1..11: note = Synthetic
QQYNSYPRALT

SEQ ID NO: 191 - protein, 11 aa, synthetic construct
  REGION 1..11: note = Synthetic
KASQNVGPTVA

SEQ ID NO: 192 - protein, 32 aa, synthetic construct
  REGION 1..32: note = Synthetic
GVPDRFTGSGSGTDFTLTISNVHSEDLAEYFC

SEQ ID NO: 193 - protein, 9 aa, synthetic construct
  REGION 1..9: note = Synthetic
QQYNSYPFT

SEQ ID NO: 194 - protein, 11 aa, synthetic construct
  REGION 1..11: note = Synthetic
FGSGTKLEIKR

SEQ ID NO: 195 - protein, 23 aa, synthetic construct
  REGION 1..23: note = Synthetic
DIQMTQTPASLSASLGDRVTISC

SEQ ID NO: 196 - protein, 11 aa, synthetic construct
  REGION 1..11: note = Synthetic
RASQDISNFLN

SEQ ID NO: 197 - protein, 15 aa, synthetic construct
  REGION 1..15: note = Synthetic
WYQQKPNGTVKLLVF

SEQ ID NO: 198 - protein, 7 aa, synthetic construct
  REGION 1..7: note = Synthetic
YTSRLHS

SEQ ID NO: 199 - protein, 32 aa, synthetic construct
  REGION 1..32: note = Synthetic
GVPSRFSGSGSGAEHSLTISNLEQEDVATYFC

SEQ ID NO: 200 - protein, 9 aa, synthetic construct
  REGION 1..9: note = Synthetic
QQGFTLPWT

SEQ ID NO: 201 - protein, 11 aa, synthetic construct
  REGION 1..11: note = Synthetic
FGGGTKVEIKR

SEQ ID NO: 202 - protein, 23 aa, synthetic construct
  REGION 1..23: note = Synthetic
DVLMTQTPLSLPVSLGDQASFSC

SEQ ID NO: 203 - protein, 16 aa, synthetic construct
  REGION 1..16: note = Synthetic
RSSQSLIHSNGNTYLH

SEQ ID NO: 204 - protein, 9 aa, synthetic construct
  REGION 1..9: note = Synthetic
SQSTHVPWT

SEQ ID NO: 205 - protein, 23 aa, synthetic construct
  REGION 1..23: note = Synthetic
DIVMTQSQKFMSTSIGDRVSVTC

SEQ ID NO: 206 - protein, 11 aa, synthetic construct
  REGION 1..11: note = Synthetic
RASQNVGPNLA

SEQ ID NO: 207 - protein, 7 aa, synthetic construct
  REGION 1..7: note = Synthetic
SASYRFS

SEQ ID NO: 208 - protein, 9 aa, synthetic construct
  REGION 1..9: note = Synthetic
QQYNRYPFT

SEQ ID NO: 209 - skipped

SEQ ID NO: 210 - protein, 17 aa, synthetic construct
  REGION 1..17: note = Synthetic
  VARIANT 7: note = where Xaa at position 7 is G or D
  VARIANT 8: note = where Xaa at position 8 is S or T or R
  VARIANT 9: note = where Xaa at position 9 is I or T
  VARIANT 13: note = where Xaa at position 13 is E or D
  VARIANT 14: note = where Xaa at position 14 is K or E
  VARIANT 16: note = where Xaa at position 16 is T or K
WIYPRDXXXKYNXXFXD

SEQ ID NO: 211 - skipped

SEQ ID NO: 212 - protein, 17 aa, synthetic construct
  REGION 1..17: note = Synthetic
  VARIANT 8: note = where Xaa at position 8 is N or I or Q or A
  VARIANT 9: note = where Xaa at position 9 is S or T
  VARIANT 17: note = where Xaa at position 17 is A or S
KSSQSLLXXRTRKNYLX

SEQ ID NO: 213 - skipped

SEQ ID NO: 214 - protein, 7 aa, synthetic construct
  REGION 1..7: note = Synthetic
  VARIANT 3: note = where Xaa at position 3 is E or D
  VARIANT 5: note = where Xaa at position 5 is M or L
GGXAXDY

SEQ ID NO: 215 - protein, 16 aa, synthetic construct
  REGION 1..16: note = Synthetic
  VARIANT 10: note = where Xaa at position 10 is D or E or A
  VARIANT 11: note = where Xaa at position 11 is G or A
  VARIANT 16: note = where Xaa at position 16 is N or S
KSSQSLLDSXXKTYLX

SEQ ID NO: 216 - protein, 9 aa, synthetic construct
  REGION 1..9: note = Synthetic
  VARIANT 8: note = where Xaa at position 8 is W or Y
WQGTHFPXT

SEQ ID NO: 217 - DNA, 342 bp, synthetic construct
  misc_feature 1..342: note = Synthetic
  source 1..342: mol_type = other DNA
caggtgcagctgaagcagtctggacctgagctggtgaagcctggggcttcagtgaagttgtcctgcaaggcttctggctacaccttcacaaccgacgatataaactgggtgaagcagaggcctggacagggacttgagtggattggatggatttatcctagagatgatagaactaagtacaatgacaagttcaaggacaaggccacattgactgtagacacatcttccaacacagcgtacatggacctccacagcctgacatctgaggactctgcggtctatttctgttcaagcctcgaggatacttactggggccaagggactctggtcgctgtctcttca

SEQ ID NO: 218 - DNA, 342 bp, synthetic construct
  misc_feature 1..342: note = Synthetic
  source 1..342: mol_type = other DNA
caggtgcagctgaagcagtctggacctgagctggtgaagcctggggcttcagtgaagttgtcctgcaaggcttctggctacaccttcacaagtaacgatataaactgggtgaagcagaggcctggacagggacttgagtggattggatggatttatcctagagatgggagtattaaatataatgagaaattcacggacaaggccacattgacagttgacgtatcctccagcacagcgtacatggagctccacagcctgacatctgaggactctgcggtctatttctgttcaggtgtcgaggattcttactggggccaagggactctggtcactgtctcttca

SEQ ID NO: 219 - DNA, 342 bp, synthetic construct
  misc_feature 1..342: note = Synthetic
  source 1..342: mol_type = other DNA
caggtgcagctgaagcagtctggacctgaactggtgaagcctggggcttcagtgaaattgtcctgcaaggcttctggctacaccttcacaagtaacgatataaactgggtgaaacagaggcctggacagggacttgagtggattggatggatttatcctagagatggtactactaagtacaatgaggagttcacggacaaggccacattgactgttgacgtatcctccagcacagcgttcatggagctccacagcctgacatctgaggactctgctgtctatttctgttcaagtgtcgaggattcttactggggccaagggactctggtcactgtctcttca

SEQ ID NO: 220 - DNA, 342 bp, synthetic construct
  misc_feature 1..342: note = Synthetic
  source 1..342: mol_type = other DNA
caggtgcagctgaagcagtctggacctgagctggtgaagcctggggcttcagtgaagttgtcctgcaaggcttctggctacaccttcacaagtaacgatataaactgggtgaagcagaggcctggacagggacttgagtggattggatggatttatcctagagatggtactactaagtacaatgagaagttcacggacaaggccacattgactgttgacgtatcctccagcacagcgttcatggagctccacaggctgacatctgaggactctgcggtctatttctgttcaagtgtcgaggattcttactggggccaagggactctggtcactgtctcttca

SEQ ID NO: 221 - DNA, 348 bp, synthetic construct
  misc_feature 1..348: note = Synthetic
  source 1..348: mol_type = other DNA
cagatccagttggtacagtctggacctgagctgaagaagcctggagagacagtcaagatctcctgcaaggcttctgggtatattttcacaagctatggaatgagctgggtgagacaggctccaggaaagggtttaaagtggatgggctggataaacacctactctggagtgccaacatatgctgatgacttcaagggacggtttgccttctctttggaaacctctgccagaactccctatttgcagatcaacaacctcaaaaatgaggacacggctacatatttctgcgcaagagggggcgaagctatggactactggggtcaaggaacctcagtcaccgtctcctca

SEQ ID NO: 222 - DNA, 348 bp, synthetic construct
  misc_feature 1..348: note = Synthetic
  source 1..348: mol_type = other DNA
cagatccagttggtacagtctggacctgagctgaagacgccaggagagacagtcaagatctcctgcaaggcttctgggtatatcttcacatcctatggaattacctgggtgaaacaggctccaggaaagggtttaaagtggatgggctggataaacacctactctggagtgccaacatatgctgatgacttcaagggacggtttgccttctctttggaaacgtctgccagcactgcctatttgcagatcaacaacctcaaaaatgaggacacgactacatatttctgtacaagagggggtgatgctttggactactggggtcaaggaacctcagtcaccgtctcctca

SEQ ID NO: 223 - DNA, 339 bp, synthetic construct
  misc_feature 1..339: note = Synthetic
  source 1..339: mol_type = other DNA
caggtgcagctgaagcagtctggagctgagctgatgaagcctggggcctcagtgaagctttcctgcaaggctactggctacacattcactggcaagtggatagagtgggtaaaacagaggcctggacatggcctagagtggattggagagattttacctggaactggtagtactaactacaatgagaagttcaagggcaaggccacattcactgcagactcatcctccaacacagcctacatgcaactcagcagcctgacaactgaagactctgctatgtattattgtttaagatccgaggatgtctggggcacagggaccacggtcaccgtctcctca

SEQ ID NO: 224 - DNA, 339 bp, synthetic construct
  misc_feature 1..339: note = Synthetic
  source 1..339: mol_type = other DNA
caggtgcagctgaagcagtctggagctgagctgatgaagcctggggcctcagtgaagcttgcctgcaaggctactggctacacattcactggctactggatagagtggataaagcagaggcctggacaaggccttgagtggattggagagatgttacctggaagtggtagtactcactacaatgagaagttcaagggtaaggccacattcactgcagatacatcctccaacacagcctacatgcaactcagcggcctgacaactgaggactctgccatctattactgtgtaagaagcatagactactggggccaaggcaccactctcacagtctcctca

SEQ ID NO: 225 - DNA, 375 bp, synthetic construct
  misc_feature 1..375: note = Synthetic
  source 1..375: mol_type = other DNA
caggtgcagctgaagcagtctgggcctgagctggcaaggccttgggcttcagtgaagatatcctgccaggctttctacaccttttccagaagggtgcactttgccattagggataccaactactggatgcagtgggtaaaacagaggcctggacagggtctggaatggatcggggctatttatcctggaaatggtgatactagttacaatcagaagttcaagggcaaggccacattgactgcagacaaatcctccagcacagcctacatgcaactcagcagcctgacatctgaggactctgcggtctattactgtgcatccggtagccactactttgactactggggccaaggcaccactctcacagtctcctca

SEQ ID NO: 226 - DNA, 369 bp, synthetic construct
  misc_feature 1..369: note = Synthetic
  source 1..369: mol_type = other DNA
gaggtccagctgcaacaatctgggcctgagctggtgaagcctggggcttcagtgaaggtatcctgtaaggcttctggatacacgctcactgactactacatgaactgggtgaagcagagccatggaaagagccttgagtggattggagatgttaatcctaacaatgatggtactacctacaaccagaaattcaagggcagggccacattgactgtagacaagtcttccaacacagcctccatggagctccgcagcctgacatctgaggactctgcagtctactactgtgcaatatgccccttttattacctcggtaaagggacccactttgactactggggccaaggcacctctctcacagtctcctca

SEQ ID NO: 227 - DNA, 372 bp, synthetic construct
  misc_feature 1..372: note = Synthetic
  source 1..372: mol_type = other DNA
gaggtccagctgcaacaatctggacctgtgctggtgaagcctggggcttcagggaagatgtcctgtaaggcttctggatacaaattcactgactactatatgatctgggtgaagcagagccatggaaagagccttgagtggattggagttattaaaatttataacggtggtacgagctacaaccagaagttcaagggcaaggccacattgactgttgacaagtcctccagcacagcctacatggagctcaacagcctgacatctgaggactctgcagtctattactgtgcaagagggccatctctctatgattacgacccttactggtacttcgatgtctggggcacagggaccacggtcaccgtctcctca

SEQ ID NO: 228 - DNA, 360 bp, synthetic construct
  misc_feature 1..360: note = Synthetic
  source 1..360: mol_type = other DNA
caggtgcagctgaagcagtctggaactgagctgatgaagcctggggcctcagtgaacctttcctgcaaggcttctggctacacattcactgcctactggatagagtgggtaaagcagaggcctggacatggccttgagtggattggagagattttacctggaagtggtactactaactacaatgagaacttcaaggacagggccacattcactgcagatacatcctccaacacagcctacatgcaactcagcagcctgacaagtgaggactctgccatctattactgtgcaagatcctattactacgctagtagatggtttgctttctggggccaagggactctggtcactgtctcttca

SEQ ID NO: 229 - DNA, 360 bp, synthetic construct
  misc_feature 1..360: note = Synthetic
  source 1..360: mol_type = other DNA
gaggtccagctgcagcagcctggggctgagcttgtgaagcctggggcttcagtgaagatgtcctgtaaggcttctggctacaccttcaccagctactggataacctgggtgaagcagaggcctggacaaggccttgagtggattggagatatttatcctggtagtggtagtactaactacaatgagaagttcaagagcaaggccacactgactgtagacacatcctccagcacagcctacatgcagctcagcagcctgacatctgaggactctgcggtctattactgtgcaagaaggagatactacgctacggcctggtttgcttactggggccaagggactctggtcactgtctcttca

SEQ ID NO: 230 - DNA, 360 bp, synthetic construct
  misc_feature 1..360: note = Synthetic
  source 1..360: mol_type = other DNA
caggtgcagctgaagcagtctggggctgagctggtgaggcctggggcttcagtgaagctgtcctgcaaggcttctggctacactttcactgactactatataaactgggtgaagcagaggcctggacagggacttgagtggattgcaaggatttatcctggaagtggtaatacttactacaatgagaagttcaagggcaaggccacactgactgcagaaaaatcctccagcactgcctacatgcagctcagcagcctgacatctgaggactctgctgtctatttctgtgcaagaaattactacattagtagtccctggtttgcttactggggccaagggactctggtcactgtctcttca

SEQ ID NO: 231 - DNA, 360 bp, synthetic construct
  misc_feature 1..360: note = Synthetic
  source 1..360: mol_type = other DNA
caggtgcagctgaagcagtctggggctgagctagtgacgcctggagcctcagtgaagatgtcctgcaaggcttctggctacaccttcactacctatcctatagagtggatgaaacagaatcatggaaagagcctagagtggattggaaattttcatccttacaatgatgatactaagtacaatgaaaagttcaagggcaaggccacattgactgtagaaaaatcctctaacacagtctacttggagctcagccgattaacatctgatgactctgctgtttatttctgtgcaaggagggtctactatagttacttctggtttggttactggggccacgggactctggtcactgtctcttca

SEQ ID NO: 232 - DNA, 360 bp, synthetic construct
  misc_feature 1..360: note = Synthetic
  source 1..360: mol_type = other DNA
caggtgcagctgaagcagtctggggctgagctagtgaaacctggagcctcagtgaagatgtcctgcaaggcttctggctacaccttcactacctatcctatagagtggatgaagcagaatcatgggaagagcctagagtggattggaaattttcatccttacaatggtgattctaagtacaatgaaaagttcaagggcaaggccaccttgactgtagaaaaatcctctagcacagtctacttagaactcagccgattaccatctgctgactctgctatttattactgtgcaaggaggcactacgctgctagtccctggtttgctcactggggccaagggactctggtcactgtctcttca

SEQ ID NO: 233 - DNA, 339 bp, synthetic construct
  misc_feature 1..339: note = Synthetic
  source 1..339: mol_type = other DNA
gacattgtgatgacccagtctccatcctccctggctgtgtcagcaggagagaaggtcactatgacctgcaaatccagtcagagtctgctcaacagtagaacccgaaagaactacttggcttggtaccagcagaaaccagggcagtctcctaaactgctgatctactgggcatccactagggaatctggggtccctgatcgcttcacaggcagtggatctgggacagatttctctctcaccatcagcagtgtgcaggctgaagacctggcagtttattactgcaagcaatcttataatctgtacacgttcggaggggggaccaagctggaaataaaacgg

SEQ ID NO: 234 - DNA, 339 bp, synthetic construct
  misc_feature 1..339: note = Synthetic
  source 1..339: mol_type = other DNA
gacattgtgatgacccagtctccatcctccctggctgtgtcagcaggagagagggtcactatgagctgcaaatccagtcagagtctgctcatcagtagaacccgaaagaactatttgtcttggtaccagcagaaaccagggcagtctcctaaactgctgatctactgggcatccactagggaatctggggtccctgatcgcttcacaggcagtggatctgggacagatttcactctcaccatcagcagtgtacaggctgaagacctggcagtttattactgcaagcaatcttataatctgtacacgttcggcggggggaccaagctggaaataaaacgg

SEQ ID NO: 235 - DNA, 339 bp, synthetic construct
  misc_feature 1..339: note = Synthetic
  source 1..339: mol_type = other DNA
gacattgtgatgacccagtctccatcctccctggctgtgtcagcaggagagaaggtcactatgagctgcaaatccagtcagagtctgctcatcagtagaacccgaaagaactatttgtcttggtaccagcagaaaccagggcagtctcctaaactgctgatctattgggcatccactagggaatctggggtccctgatcgcttcacaggcagtggatctgggacagatttcactctcaccatcagcagtgtacaggctgaagacctggcagtttattactgcaaacaatcttataatctgtacacgttcggcggggggaccaagctggaaatcaaacgg

SEQ ID NO: 236 - DNA, 339 bp, synthetic construct
  misc_feature 1..339: note = Synthetic
  source 1..339: mol_type = other DNA
gatgttttgatgacccaaactccactcactttgtcggttaccattggacaaccagcctccatctcttgcaagtcaagtcagagcctcttagatagtgatggaaagacatatttgaattggttgttacagaggccaggccagtctccaaagcgcctaatctatctggtgtctaaactggactctggagtccctgacaggttcactggcagtggatcagggacagatttcacactgaaaatcagcagagtggaggctgaggatttgggagtttattattgctggcaaggtacacattttccgtggacgttcggtggaggcaccaagctggaaatcaaacgg

SEQ ID NO: 237 - DNA, 339 bp, synthetic construct
  misc_feature 1..339: note = Synthetic
  source 1..339: mol_type = other DNA
gatattgtgatgacgcaggctccactcactttgtcggttaccattggacaaccagcctccatctcttgcaagtcaagtcagagcctcttagatagtgatggaaagacatatttgagttggttgttacagaggccaggccagtctccaaagcgcctaatctatctggtgtctaaactggactctggagtccctgacaggttcactggcagtggatcagggacagatttcacactgaaaatcagcagagtggaggctgaggatttgggagtttattattgctggcaaggtacacattttccgtacacgttcggaggggggaccaagctggaaataaaacgg

SEQ ID NO: 238 - DNA, 339 bp, synthetic construct
  misc_feature 1..339: note = Synthetic
  source 1..339: mol_type = other DNA
gacattgtgatgacccagtctccatcctccctggctgtgtcagcaggagagaaggtcactatgagctgcaaatccagtcagagtctgctcaacagtagaacccgaaagaactacttggcttggtaccagcagaaaccagggcagtctcctaaactgctgatctactgggcatccactagggaatctggggtccctgatcgcttcacaggcagtggatctggaacagatttcactctcaccatcagcagtgtgcaggctgaagacctggcagtttattactgcaagcaatcttataatattccgacgttcggtggaggcaccaagctggaaatcaaacgg

SEQ ID NO: 239 - DNA, 339 bp, synthetic construct
  misc_feature 1..339: note = Synthetic
  source 1..339: mol_type = other DNA
gatgttttgatgacccaaactccactctccctgcctgtcagtcttggagaacaagcctccatctcttgcagatcaagtcagagccttgtacaaagtaatggaaacacctatttacattggtacctgcagaagccaggccagtctccaaagctcctgatctacaaagtttccaaccgattttctggggtcccagacaggttcagtggcagtggatcagggacagatttcacactcaagatcagcagagtggaggctgaggatctgggagtttatttctgctctcaaagtacacatgttcctccgacgttcggtggaggcaccaagctggaaatcaaacgg

SEQ ID NO: 240 - DNA, 324 bp, synthetic construct
  misc_feature 1..324: note = Synthetic
  source 1..324: mol_type = other DNA
gacatccagctgactcagtctccagccatcctgtctgtgagtccaggagaaagagtcagtttctcctgcagggccagtcagagcattggcacaagcatacactggtatcagcaaagaacaaatggttctccaaggcttctcataaagtatgcttctgagtctatctctgggatcccttccaggtttagtggcagtggatcagggacagattttactcttagcatcaacagtgtggagtctgaagatattgcagattattactgtcaacaaagtaatagctggccgtacacgttcggaggggggaccaagctggaaataaaacgg

SEQ ID NO: 241 - DNA, 324 bp, synthetic construct
  misc_feature 1..324: note = Synthetic
  source 1..324: mol_type = other DNA
gatatccagatgacacagactccagcctccctgtctgcctctctgggagacagagtcaccatcagttgtagggcaagtcaggacattagcaattttttaaactggtatcaacagaaaccgaatggaactgttaaactcctagtcttctacacatcaagattacactcaggagtcccatcaaggttcagtggcagtgggtctggagcagagcattctctcaccattagcaacctggagcaggaagatgttgccacttacttttgccaacagggttttacgcttccgtggacgttcggtgggggcaccaaggtggaaatcaaacgg

SEQ ID NO: 242 - DNA, 339 bp, synthetic construct
  misc_feature 1..339: note = Synthetic
  source 1..339: mol_type = other DNA
gatgttttgatgacccaaactccactctccctgcctgtcagtcttggagatcaagcctccttctcttgcagatctagtcagagccttatacacagtaatggaaacacctatttacattggtacctgcagaagccaggccagtctccaaagctcctgatctacaaagtttccaaccgattttctggggtcccagacaggttcagtggcagtggatcagggacagatttcacactcaagatcagcagagtggaggctgaggatctgggagtttatttctgctctcaaagtacacatgttccgtggacgttcggtggaggcaccaagctggaaatcaaacgg

SEQ ID NO: 243 - DNA, 324 bp, synthetic construct
  misc_feature 1..324: note = Synthetic
  source 1..324: mol_type = other DNA
gacattgtgatgacccagtctcaaaaattcatgtccacatcaataggagacagggtcagcgtcacctgcagggccagtcagaatgtgggtcccaatttagcctggtatcaacagaaaccagggcaatctcctaaagcactgatttactcggcatcctaccgattcagtggagtccctgatcgcttcacaggcagtggatctgggacagatttcactctcaccatcagcaatgtgcagtctgaagacttggcagagtatttctgtcagcaatataacaggtatccattcacgttcggctcggggacaaagttggaaataaaacgg

SEQ ID NO: 244 - DNA, 324 bp, synthetic construct
  misc_feature 1..324: note = Synthetic
  source 1..324: mol_type = other DNA
gacattgtgatgacccagtctcaaaaattcatgtccacatcagtaggagacagggtcagcatcacctgcaaggccagtcagaatgtgggtactgctgtagcctggtatcaacagaaaccaggacaatctcctaaactactgatttcctcggcatccaatcggtacactggagtccctgatcgcttcacaggcagtggatctgggacagatttcactctcaccatcagtaatatgcagtctgaagacgtggcagattatttctgccagcaatataacagctatcctctcacgttcggtgctgggaccaagctggagctgaaacgg

SEQ ID NO: 245 - DNA, 324 bp, synthetic construct
  misc_feature 1..324: note = Synthetic
  source 1..324: mol_type = other DNA
gacattgtgatgacccagtctcaaaaattcatgtccacttcagtaggagacagggtcagcgtcacctgcaaggccagtcagaatgtgggtcctaatgtagcctggtatcaacagaaaccagggcaatctcctaaagcactgatttactcggcatcctaccggtacagtggagtccctgatcgcttcacaggcagtggatctgggacagatttcactctcaccatcagcaatgtgcagtctgaagacttggcagactatttctgtcagcaatataaccgctatcctctcacgttcggtgctgggaccaaactggagctgaaacgg

SEQ ID NO: 246 - DNA, 330 bp, synthetic construct
  misc_feature 1..330: note = Synthetic
  source 1..330: mol_type = other DNA
gacattgtgatgacccagtctcaaaaattcatgtccacatcagtaggagacagggtcaacgtcacctgcaaggccagtcagaatgtgggtactcatgtagcctggtatcaacagaaaccagggcaatctcctaaagcactgatttactcggcatcctaccggtacagtggcgtccctgatcgcttcacaggcagtggatctgggacagatttcactctcaccatcagcaatgtgcagtctgaagacctggcagagtatttctgtcagcaatataacagctatcctcgagcgctcacgttcggtgctgggaccaagctggagctgaaacgg

SEQ ID NO: 247 - DNA, 324 bp, synthetic construct
  misc_feature 1..324: note = Synthetic
  source 1..324: mol_type = other DNA
gacattgtgatgacccagtctcaaaaattcatgtccacatcagtaggagacagggtcaacgtcacctgcaaggccagtcagaatgtgggtcctactgtagcctggtatcaacagaaaccagggcaatctcctaaagcactaatttactcggcatcctaccggtacagtggagtccctgatcgcttcacaggcagtggatctgggacagatttcactctcaccatcagcaatgtgcactctgaagacttggcagagtatttctgtcagcaatataacagctatccattcacgttcggctcggggacaaagttggaaataaaacgg

SEQ ID NO: 248 - protein, 114 aa, synthetic construct
  REGION 1..114: note = Synthetic
QVQLVQSGAEVKKPGASVKVSCKASGYTFTTDDINWVRQAPGQGLEWIGWIYPRDDRTKYNDKFKDKATLTVDTSSNTAYMELSSLRSEDTAVYYCSSLEDTYWGQGTLVTVSS

SEQ ID NO: 249 - protein, 114 aa, synthetic construct
  REGION 1..114: note = Synthetic
QVQLVQSGAEVKKPGASVKVSCKASGYTFTTDDINWVRQAPGQGLEWIGWIYPRDDRTKYNDKFKDRATLTVDTSSNTAYMELSSLRSEDTAVYYCSSLEDTYWGQGTLVTVSS

SEQ ID NO: 250 - protein, 113 aa, synthetic construct
  REGION 1..113: note = Synthetic
DIVMTQSPDSLAVSLGERATINCKSSQSLLNSRTRKNYLAWYQQKPGQPPKLLIYWASTRESGVPDRFSGSGSGTDFTLTISSLQAEDVAVYYCKQSYNLYTFGQGTKVEIKR

SEQ ID NO: 251 - protein, 116 aa, synthetic construct
  REGION 1..116: note = Synthetic
QIQLVQSGSELKKPGASVKVSCKASGYIFTSYGMSWVRQAPGKGLKWMGWINTYSGVPTYADDFKGRFVFSLDTSVRTPYLQISSLKAEDTAVYFCARGGEAMDYWGQGTLVTVSS

SEQ ID NO: 252 - protein, 116 aa, synthetic construct
  REGION 1..116: note = Synthetic
QIQLVQSGSELKKPGASVKVSCKASGYIFTSYGMSWVRQAPGKGLKWMGWINTYSGVPTYADDFKGRFVFSLDTSVRTPYLQISSLKAEDTATYFCARGGEAMDYWGQGTLVTVSS

SEQ ID NO: 253 - protein, 113 aa, synthetic construct
  REGION 1..113: note = Synthetic
DVLMTQTPLSLSVTPGQPASISCKSSQSLLDSDGKTYLNWLLQRPGQSPKRLIYLVSKLDSGVPDRFSGSGSGTDFTLKISRVEAEDVGVYYCWQGTHFPWTFGQGTKVEIKR

SEQ ID NO: 254 - protein, 113 aa, synthetic construct
  REGION 1..113: note = Synthetic
QVQLVQSGAEVKKPGASVKVSCKASGYTFTGKWIEWVRQAPGQGLEWIGEILPGTGSTNYAQKFQGRATFTADSSTSTAYMELSSLRSEDTAVYYCLRSEDVWGQGTLVTVSS

SEQ ID NO: 255 - protein, 113 aa, synthetic construct
  REGION 1..113: note = Synthetic
QVQLVQSGAEVKKPGASVKVSCKASGYTFTGKWIEWVRQAPGQGLEWIGEILPGTGSTNYNEKFKGRATFTADSSTSTAYMELSSLRSEDTAVYYCLRSEDVWGQGTLVTVSS

SEQ ID NO: 256 - protein, 113 aa, synthetic construct
  REGION 1..113: note = Synthetic
DIVMTQSPDSLAVSLGERATINCKSSQSLLNSRTRKNYLAWYQQKPGQPPKLLIYWASTRESGVPDRFSGSGSGTDFTLTISSLQAEDVAVYYCKQSYNIPTFGQGTKVEIKR

SEQ ID NO: 257 - protein, 17 aa, synthetic construct
  REGION 1..17: note = Synthetic
KSSQSLLQSRTRKNYLA

SEQ ID NO: 258 - protein, 17 aa, synthetic construct
  REGION 1..17: note = Synthetic
KSSQSLLASRTRKNYLA

SEQ ID NO: 259 - protein, 17 aa, synthetic construct
  REGION 1..17: note = Synthetic
KSSQSLLNTRTRKNYLA

SEQ ID NO: 260 - protein, 17 aa, synthetic construct
  REGION 1..17: note = Synthetic
  VARIANT 8: note = wherein Xaa at position 8 is N or Q or A
  VARIANT 9: note = where Xaa at position 9 is S or T
KSSQSLLXXRTRKNYLA

SEQ ID NO: 261 - protein, 16 aa, synthetic construct
  REGION 1..16: note = Synthetic
KSSQSLLDSEGKTYLN

SEQ ID NO: 262 - protein, 16 aa, synthetic construct
  REGION 1..16: note = Synthetic
KSSQSLLDSAGKTYLN

SEQ ID NO: 263 - protein, 16 aa, synthetic construct
  REGION 1..16: note = Synthetic
KSSQSLLDSDAKTYLN

SEQ ID NO: 264 - protein, 30 aa, synthetic construct
  REGION 1..30: note = Synthetic
QVQLVQSGAEVKKPGASVKVSCKASGYTFT

SEQ ID NO: 265 - protein, 14 aa, synthetic construct
  REGION 1..14: note = Synthetic
WVRQAPGQGLEWIG

SEQ ID NO: 266 - protein, 32 aa, synthetic construct
  REGION 1..32: note = Synthetic
KATLTVDTSSNTAYMELSSLRSEDTAVYYCSS

SEQ ID NO: 267 - protein, 32 aa, synthetic construct
  REGION 1..32: note = Synthetic
RATLTVDTSSNTAYMELSSLRSEDTAVYYCSS

SEQ ID NO: 268 - protein, 11 aa, synthetic construct
  REGION 1..11: note = Synthetic
WGQGTLVTVSS

SEQ ID NO: 269 - protein, 30 aa, synthetic construct
  REGION 1..30: note = Synthetic
QIQLVQSGSELKKPGASVKVSCKASGYIFT

SEQ ID NO: 270 - protein, 32 aa, synthetic construct
  REGION 1..32: note = Synthetic
RFVFSLDTSVRTPYLQISSLKAEDTAVYFCAR

SEQ ID NO: 271 - protein, 32 aa, synthetic construct
  REGION 1..32: note = Synthetic
RFVFSLDTSVRTPYLQISSLKAEDTATYFCAR

SEQ ID NO: 272 - protein, 11 aa, synthetic construct
  REGION 1..11: note = Synthetic
WGQGTLVTVSS

SEQ ID NO: 273 - protein, 30 aa, synthetic construct; identical to SEQ ID NO: 264
  REGION 1..30: note = Synthetic

SEQ ID NO: 274 - protein, 14 aa, synthetic construct
  REGION 1..14: note = Synthetic
WVRQAPGQGLEWIG

SEQ ID NO: 275 - protein, 17 aa, synthetic construct
  REGION 1..17: note = Synthetic
EILPGTGSTNYAQKFQG

SEQ ID NO: 276 - protein, 32 aa, synthetic construct
  REGION 1..32: note = Synthetic
RATFTADSSTSTAYMELSSLRSEDTAVYYCLR

SEQ ID NO: 277 - protein, 11 aa, synthetic construct
  REGION 1..11: note = Synthetic
WGQGTLVTVSS

SEQ ID NO: 278 - protein, 113 aa, synthetic construct
  REGION 1..113: note = Synthetic
DIVMTQSPDSLAVSLGERATINCKSSQSLLASRTRKNYLAWYQQKPGQPPKLLIYWASTRESGVPDRFSGSGSGTDFTLTISSLQAEDVAVYYCKQSYNLYTFGQGTKVEIKR

SEQ ID NO: 279 - protein, 113 aa, synthetic construct
  REGION 1..113: note = Synthetic
DVLMTQTPLSLSVTPGQPASISCKSSQSLLDSDAKTYLNWLLQRPGQSPKRLIYLVSKLDSGVPDRFSGSGSGTDFTLKISRVEAEDVGVYYCWQGTHFPWTFGQGTKVEIKR

SEQ ID NO: 280 - protein, 113 aa, synthetic construct
  REGION 1..113: note = Synthetic
DIVMTQSPDSLAVSLGERATINCKSSQSLLASRTRKNYLAWYQQKPGQPPKLLIYWASTRESGVPDRFSGSGSGTDFTLTISSLQAEDVAVYYCKQSYNIPTFGQGTKVEIKR

SEQ ID NO: 281 - protein, 23 aa, synthetic construct
  REGION 1..23: note = Synthetic
DIVMTQSPDSLAVSLGERATINC

SEQ ID NO: 282 - protein, 15 aa, synthetic construct
  REGION 1..15: note = Synthetic
WYQQKPGQPPKLLIY

SEQ ID NO: 283 - protein, 32 aa, synthetic construct
  REGION 1..32: note = Synthetic
GVPDRFSGSGSGTDFTLTISSLQAEDVAVYYC

SEQ ID NO: 284 - protein, 11 aa, synthetic construct
  REGION 1..11: note = Synthetic
FGQGTKVEIKR

SEQ ID NO: 285 - protein, 23 aa, synthetic construct
  REGION 1..23: note = Synthetic
DVLMTQTPLSLSVTPGQPASISC

SEQ ID NO: 286 - protein, 32 aa, synthetic construct
  REGION 1..32: note = Synthetic
GVPDRFSGSGSGTDFTLKISRVEAEDVGVYYC

SEQ ID NO: 287 - protein, 11 aa, synthetic construct
  REGION 1..11: note = Synthetic
FGQGTKVEIKR

SEQ ID NO: 288 - DNA, 342 bp, synthetic construct
  misc_feature 1..342: note = Synthetic
  source 1..342: mol_type = other DNA
caagtccaactcgtccagtccggggccgaagtcaagaagccgggagcctcagtgaaagtgtcgtgcaaagcttccggctacaccttcaccaccgatgacattaactgggtcagacaggcgcccggacaggggctggaatggatcggttggatctaccctcgggacgaccggactaagtacaacgacaagttcaaggacaaagcgaccctcaccgtcgacaccagcagcaacactgcctacatggaactgtcatccctgaggagcgaggacactgccgtgtattactgttcgagcctggaggatacctactggggacagggcactcttgtgaccgtgtcctcc

SEQ ID NO: 289 - DNA, 342 bp, synthetic construct
  misc_feature 1..342: note = Synthetic
  source 1..342: mol_type = other DNA
caagtccaactcgtccagtccggggccgaagtcaagaagccgggagcctcagtgaaagtgtcgtgcaaagcttccggctacaccttcaccaccgatgacattaactgggtcagacaggcgcccggacaggggctggaatggatcggttggatctaccctcgggacgaccggactaagtacaacgacaagttcaaggacagagcgaccctcaccgtcgacaccagcagcaacactgcctacatggaactgtcatccctgaggagcgaggacactgccgtgtattactgttcgagcctggaggatacctactggggacagggcactcttgtgaccgtgtcctcc

SEQ ID NO: 290 - DNA, 348 bp, synthetic construct
  misc_feature 1..348: note = Synthetic
  source 1..348: mol_type = other DNA
caaatccagctggtccagtccggttccgagctcaagaagccgggagcctcagtgaaagtgtcgtgcaaggcctccggttacatcttcacctcctacggaatgtcgtgggtccgccaagcacctggaaagggccttaagtggatggggtggatcaacacctatagcggcgtgcccacttacgccgacgactttaagggccggttcgtgttctccctggatacgtccgtgcgcactccgtacctccaaattagcagcctgaaggccgaagatactgcggtgtacttctgcgctagaggaggggaagccatggactactggggacagggcaccctggtcaccgtgtcgtcc

SEQ ID NO: 291 - DNA, 348 bp, synthetic construct
  misc_feature 1..348: note = Synthetic
  source 1..348: mol_type = other DNA
caaatccagctggtccagtccggttccgagctcaagaagccgggagcctcagtgaaagtgtcgtgcaaggcctccggttacatcttcacctcctacggaatgtcgtgggtccgccaagcacctggaaagggccttaagtggatggggtggatcaacacctatagcggcgtgcccacttacgccgacgactttaagggccggttcgtgttctccctggatacgtccgtgcgcactccgtacctccaaattagcagcctgaaggccgaagatactgcgacgtacttctgcgctagaggaggggaagccatggactactggggacagggcaccctggtcaccgtgtcgtcc

SEQ ID NO: 292 - DNA, 339 bp, synthetic construct
  misc_feature 1..339: note = Synthetic
  source 1..339: mol_type = other DNA
caagtccaactcgtgcagtcaggagcagaagtcaagaagccgggagcctccgtgaaagtgtcgtgcaaggcctccggatacactttcaccgggaagtggattgaatgggtccgccaggcgcccggccagggcctggagtggatcggagagatcctgcctggtaccggtagcactaactacgctcagaagttccagggcagagcgaccttcaccgccgactcgagcacctccactgcgtacatggaactgagctccctgaggtcggaggacaccgccgtgtattactgcctccggtccgaagatgtctggggccaggggaccctcgtgactgtgtcatcc

SEQ ID NO: 293 - DNA, 339 bp, synthetic construct
  misc_feature 1..339: note = Synthetic
  source 1..339: mol_type = other DNA
caagtccaactcgtgcagtcaggagcagaagtcaagaagccgggagcctccgtgaaagtgtcgtgcaaggcctccggatacactttcaccgggaagtggattgaatgggtccgccaggcgcccggccagggcctggagtggatcggagagatcctgcctggtaccggtagcactaactacaacgagaagttcaagggcagagcgaccttcaccgccgactcgagcacctccactgcgtacatggaactgagctccctgaggtcggaggacaccgccgtgtattactgcctccggtccgaagatgtctggggccaggggaccctcgtgactgtgtcatcc

SEQ ID NO: 294 - DNA, 339 bp, synthetic construct
  misc_feature 1..339: note = Synthetic
  source 1..339: mol_type = other DNA
gatattgtcatgacccagtcccccgattcccttgctgtctccctgggcgaacgcgcgactattaactgcaagagctcacagtcgctgctgaattcccggactcggaagaactacctggcctggtaccagcagaagcctgggcaaccgccgaagctcttgatctactgggcctcgactagagagagcggagtgccagaccgcttctccggttccggatcaggaaccgactttaccctgaccatctcgagcctgcaagcagaggacgtggccgtgtattactgcaagcagtcctacaacctctacacgttcggccagggcaccaaagtggaaatcaagagg

SEQ ID NO: 295 - DNA, 339 bp, synthetic construct
  misc_feature 1..339: note = Synthetic
  source 1..339: mol_type = other DNA
gatatcgtcatgacccaatcccccgattcccttgctgtctcactgggagaaagagccaccatcaactgcaagagctcgcagtccctgctggctagcaggactcgcaagaactacctggcctggtatcagcagaagcccggacagcctccaaagctcttgatctactgggcctccactcgggagtccggcgtgccggaccggttcagcggatcaggctccggtactgacttcaccctcaccatttcgtcgctgcaagcagaggacgtggcggtgtactactgcaagcagtcctacaacattccgacgtttgggcagggcaccaaagtggaaatcaagcgc

SEQ ID NO: 296 - DNA, 339 bp, synthetic construct
  misc_feature 1..339: note = Synthetic
  source 1..339: mol_type = other DNA
gacgtgctgatgacccaaacccccctttccctgtccgtgactcctggacaacccgcgtcaatctcctgcaagagctcgcagtccctcctcgactccgacggaaaaacctacctgaactggcttttgcagaggccagggcagagcccgaagcggctgatctacctcgtgtccaagctggactccggagtgccggatcgcttctcgggatcaggctcgggtaccgatttcacgctgaagatctccagagtggaagccgaggacgtgggcgtctactactgttggcagggcactcactttccgtggaccttcggtcaagggaccaaggtcgagattaagagg

SEQ ID NO: 297 - DNA, 339 bp, synthetic construct
  misc_feature 1..339: note = Synthetic
  source 1..339: mol_type = other DNA
gacgtgctgatgacccaaacccccctttccctgtccgtgactcctggacaacccgcgtcaatctcctgcaagagctcgcagtccctcctcgactccgacgcaaaaacctacctgaactggcttttgcagaggccagggcagagcccgaagcggctgatctacctcgtgtccaagctggactccggagtgccggatcgcttctcgggatcaggctcgggtaccgatttcacgctgaagatctccagagtggaagccgaggacgtgggcgtctactactgttggcagggcactcactttccgtggaccttcggtcaagggaccaaggtcgagattaagagg

SEQ ID NO: 298 - DNA, 339 bp, synthetic construct
  misc_feature 1..339: note = Synthetic
  source 1..339: mol_type = other DNA
gatatcgtcatgacccaatcccccgattcccttgctgtctcactgggagaaagagccaccatcaactgcaagagctcgcagtccctgctgaatagcaggactcgcaagaactacctggcctggtatcagcagaagcccggacagcctccaaagctcttgatctactgggcctccactcgggagtccggcgtgccggaccggttcagcggatcaggctccggtactgacttcaccctcaccatttcgtcgctgcaagcagaggacgtggcggtgtactactgcaagcagtcctacaacattccgacgtttgggcagggcaccaaagtggaaatcaagcgc

SEQ ID NO: 299 - DNA, 339 bp, synthetic construct
  misc_feature 1..339: note = Synthetic
  source 1..339: mol_type = other DNA
gatattgtcatgacccagtcccccgattcccttgctgtctccctgggcgaacgcgcgactattaactgcaagagctcacagtcgctgctggcttcccggactcggaagaactacctggcctggtaccagcagaagcctgggcaaccgccgaagctcttgatctactgggcctcgactagagagagcggagtgccagaccgcttctccggttccggatcaggaaccgactttaccctgaccatctcgagcctgcaagcagaggacgtggccgtgtattactgcaagcagtcctacaacctctacacgttcggccagggcaccaaagtggaaatcaagagg

SEQ ID NO: 300 - protein, 125 aa, synthetic construct
  REGION 1..125: note = Synthetic
AVTLDESGGGLQTPGGALSLVCKASGFTFSSNAMGWVRQAPGKGLEWVAGIDDDGSGTRYAPAVKGRATISRDNGQSTLRLQLNNLRAEDTGTYYCTKCAYSSGCDYEGGYIDAWGHGTEVIVSS

SEQ ID NO: 301 - protein, 118 aa, synthetic construct
  REGION 1..118: note = Synthetic
AVTLDESGGGLQTPGGGLSLVCKASGFTFSSYAMGWMRQAPGKGLEYVAGIRSDGSFTLYATAVKGRATISRDNGQSTVRLQLNNLRAEDTATYFCTRSGNVGDIDAWGHGTEVIVSS

SEQ ID NO: 302 - protein, 128 aa, synthetic construct
  REGION 1..128: note = Synthetic
AVTLDESGGGLQTPGGGLSLVCKASGFDFSSYQMNWIRQAPGKGLEFVAAINRFGNSTGHGAAVKGRVTISRDDGQSTVRLQLSNLRAEDTATYYCAKGVYGYCGSYSCCGVDTIDAWGHGTEVIVSS

SEQ ID NO: 303 - protein, 107 aa, synthetic construct
  REGION 1..107: note = Synthetic
ALTQPASVSANLGGTVKITCSGGGSYAGSYYYGWYQQKSPGSAPVTVIYDNDKRPSDIPSRFSGSLSGSTNTLTITGVRADDEAVYFCGSADNSGAAFGAGTTLTVL

SEQ ID NO: 304 - protein, 108 aa, synthetic construct
  REGION 1..108: note = Synthetic
ALTQPASVSANPGETVKITCSGGYSGYAGSYYYGWYQQKAPGSAPVTLIYYNNKRPSDIPSRFSGSLSGSTNTLTITGVRADDEAVYFCGSADNSGAAFGAGTTLTVL

SEQ ID NO: 305 - protein, 107 aa, synthetic construct
  REGION 1..107: note = Synthetic
ALTQPASVSANPGETVKITCSGGGSYAGSYYYGWYQQKAPGSAPVTLIYYNNKRPSDIPSRFSGSLSGSTNTLTITGVRADDEAVYFCGSADNSGAAFGAGTTLTVL

SEQ ID NO: 306 - protein, 126 aa, synthetic construct
  REGION 1..126: note = Synthetic
AVTLDESGGGLQTPGGALSLVCKASGFTFSSYAMHWVRQAPGKGLEWVAGIYKSGAGTNYAPAVKGRATISRDNGQSTVRLQLNNLRAEDTGTYYCAKTTGSGCSSGYRAEYIDAWGHGTEVIVSS

SEQ ID NO: 307 - protein, 107 aa, synthetic construct; identical to SEQ ID NO: 305
  REGION 1..107: note = Synthetic

SEQ ID NO: 308 - protein, 126 aa, synthetic construct
  REGION 1..126: note = Synthetic
AVTLDESGGGLQTPGGALSLVCKASGFTFSSYDMVWVRQAPGKGLEFVAGISRNDGRYTEYGSAVKGRATISRDNGQSTVRLQLNNLRAEDTATYYCARDAGGSAYWFDAGQIDAWGHGTEVIVSS

SEQ ID NO: 309 - protein, 107 aa, synthetic construct; identical to SEQ ID NO: 305
  REGION 1..107: note = Synthetic

SEQ ID NO: 310 - protein, 327 aa, synthetic construct
  REGION 1..327: note = Synthetic
ASTKGPSVFPLAPCSRSTSESTAALGCLVKDYFPEPVTVSWNSGALTSGVHTFPAVLQSSGLYSLSSVVTVPSSSLGTKTYTCNVDHKPSNTKVDKRVESKYGPPCPSCPAPEFLGGPSVFLFPPKPKDTLMISRTPEVTCVVVDVSQEDPEVQFNWYVDGVEVHNAKTKPREEQFNSTYRVVSVLTVLHQDWLNGKEYKCKVSNKGLPSSIEKTISKAKGQPREPQVYTLPPSQEEMTKNQVSLTCLVKGFYPSDIAVEWESNGQPENNYKTTPPVLDSDGSFFLYSRLTVDKSRWQEGNVFSCSVMHEALHNHYTQKSLSLSLGK

SEQ ID NO: 311 - protein, 327 aa, synthetic construct
  REGION 1..327: note = Synthetic
ASTKGPSVFPLAPCSRSTSESTAALGCLVKDYFPEPVTVSWNSGALTSGVHTFPAVLQSSGLYSLSSVVTVPSSSLGTKTYTCNVDHKPSNTKVDKRVESKYGPPCPPCPAPEFLGGPSVFLFPPKPKDTLMISRTPEVTCVVVDVSQEDPEVQFNWYVDGVEVHNAKTKPREEQFNSTYRVVSVLTVLHQDWLNGKEYKCKVSNKGLPSSIEKTISKAKGQPREPQVYTLPPSQEEMTKNQVSLTCLVKGFYPSDIAVEWESNGQPENNYKTTPPVLDSDGSFFLYSRLTVDKSRWQEGNVFSCSVMHEALHNHYTQKSLSLSLGK

SEQ ID NO: 312 - protein, 327 aa, synthetic construct
  REGION 1..327: note = Synthetic
ASTKGPSVFPLAPCSRSTSESTAALGCLVKDYFPEPVTVSWNSGALTSGVHTFPAVLQSSGLYSLSSVVTVPSSSLGTKTYTCNVDHKPSNTKVDKRVESKYGPPCPPCPAPEFLGGPSVFLFPPKPKDTLMISRTPEVTCVVVDVSQEDPEVQFNWYVDGVEVHNAKTKPREEQFNSTYRVVSVLTVLHQDWLNGKEYKCKVSNKGLPSSIEKTISKAKGQPREPQVYTLPPSQEEMTKNQVSLTCLVKGFYPSDIAVEWESNGQPENNYKTTPPVLDSDGSFFLYSRLTVDKSRWQEGNVFSCSVLHEALHSHYTQKSLSLSLGK

SEQ ID NO: 313 - protein, 106 aa, synthetic construct
  REGION 1..106: note = Synthetic
TVAAPSVFIFPPSDEQLKSGTASVVCLLNNFYPREAKVQWKVDNALQSGNSQESVTEQDSKDSTYSLSSTLTLSKADYEKHKVYACEVTHQGLSSPVTKSFNRGEC